European Patent Application EP 4 566 620 A1, published June 11, 2025. Title: Switchable universal chimeric antigen receptors and their use. Applicant: AvenCell Europe GmbH. Application EP. The sequence listing filed with the application follows.

SEQUENCE LISTING (197 sequences)

SEQ ID NO: 1 - protein, 33 aa, Saccharomyces cerevisiae
RMKQLEPKVEELLPKNYHLENEVARLKKLVGER

SEQ ID NO: 2 - protein, 14 aa, Saccharomyces cerevisiae
NYHLENEVARLKKL

SEQ ID NO: 3 - protein, 51 aa, Homo sapiens
MDPDLEIRAAFLRQRNTALRTEVAELEQEVQRLENEVSQYETRYGPLGGGK

SEQ ID NO: 4 - protein, 51 aa, Homo sapiens
MDPDLEIEAAFLERENTALETRVAELRQRVQRLRNRVSQYRTRYGPLGGGK

SEQ ID NO: 5 - protein, 10 aa, Homo sapiens
KPLPEVTDEY

SEQ ID NO: 6 - protein, 20 aa, Homo sapiens
  VARIANT 16: note = Xaa can be any naturally occuring amino acid
LEKEALKKIIEDQQEXLNKW

SEQ ID NO: 7 - protein, 20 aa, Homo sapiens
LEKEALKKIIEDQQEALNKW

SEQ ID NO: 8 - protein, 8 aa, synthetic construct
  source 1..8: note = humanized CDR sequence
GYTFTHYY

SEQ ID NO: 9 - protein, 8 aa, synthetic construct
  source 1..8: note = humanized CDR sequence
VNPSNGGT

SEQ ID NO: 10 - protein, 13 aa, synthetic construct
  source 1..13: note = humanized CDR sequence
ARSEYDYGLGFAY

SEQ ID NO: 11 - protein, 12 aa, synthetic construct
  source 1..12: note = humanized CDR sequence
QSLLNSRTPKNY

SEQ ID NO: 12 - protein, 8 aa, synthetic construct
  source 1..8: note = humanized CDR sequence
KQSYNLLT

SEQ ID NO: 13 - protein, 113 aa, synthetic construct
  source 1..113: note = humanized scFv VL chain
  VARIANT 24: note = Xaa can be any naturally occurring amino acid
  VARIANT 35: note = Xaa can be any naturally occurring amino acid
  VARIANT 61: note = Xaa can be any naturally occurring amino acid
  VARIANT 101: note = Xaa can be any naturally occurring amino acid
DIVMTQSPDSLAVSLGERATINCXSSQSLLNSRTXKNYLAWYQQKPGQPPKLLIYWASTRXSGVPDRFSGSGSGTDFTLTISSLQAEDVAVYYCKQSYNLXTFGGGTKVEILK

SEQ ID NO: 14 - protein, 112 aa, synthetic construct
  source 1..112: note = humanized scFv VL chain
DIVMTQSPDSLAVSLGERATINCKSSQSLLNSRTPKNYLAWYQQKPGQPPKLLIYWASTRKSGVPDRFSGSGSGTDFTLTISSLQAEDVAVYYCKQSYNLLTFGGGTKVEIK

SEQ ID NO: 15 - protein, 120 aa, synthetic construct
  source 1..120: note = humanized scFv VL chain
QVQLVQSGAEVKKPGASVKVSCKASGYTFTHYYIYWVRQAPGQGLEWMGGVNPSNGGTHFNEKFKSRVTMTRDTSISTAYMELSRLRSDDTAVYYCARSEYDYGLGFAYWGQGTLVTVSS

SEQ ID NO: 16 - protein, 112 aa, synthetic construct
  source 1..112: note = humanized scFv VL chain
DIVMTQSPDSLAVSLGERATINCRSSQSLLDSRTKKNYLAWYQQKPGQPPKLLIYWASTRESGVPDRFSGSGSGTDFTLTISSLQAEDVAVYYCKQSYNLPTFGGGTKVEIK

SEQ ID NO: 17 - protein, 118 aa, synthetic construct
  source 1..118: note = humanized scFv VH chain
EVQLVESGGGLVQPGGSLRLSCAASGFTFSDFWMNWVRQAPGKGLEWVGQIRNKPNNYETYYSDSLKGRFTISRDDSKSITYLQMNSLRAEDTAVYYCTLGNSWFAYWGQGTLVTVSS

SEQ ID NO: 18 - protein, 219 aa, synthetic construct
  source 1..219: note = humanized Fab fragment
GQVQLVQSGAEVKKPGASVKVSCKASGYTFTHYYIYWVRQAPGQGLEWMGGVNPSNGGTHFNEKFKSRVTMTRDTSISTAYMELSRLRSDDTAVYYCARSEYDYGLGFAYWGQGTLVTVSSASTKGPSVFPLAPSSKSTSGGTAALGCLVKDYFPEPVTVSWNSGALTSGVHTFPAVLQSSGLYSLSSVVTVPSSSLGTQTYICNVNHKPSNTKVDKKV

SEQ ID NO: 19 - protein, 219 aa, synthetic construct
  source 1..219: note = humanized Fab fragment
DIVMTQSPDSLAVSLGERATINCKSSQSLLNSRTPKNYLAWYQQKPGQPPKLLIYWASTRKSGVPDRFSGSGSGTDFTLTISSLQAEDVAVYYCKQSYNLLTFGGGTKVEIKRTVAAPSVFIFPPSDEQLKSGTASVVCLLNNFYPREAKVQWKVDNALQSGNSQESVTEQDSKDSTYSLSSTLTLSKADYEKHKVYACEVTHQGLSSPVTKSFNRGEC

SEQ ID NO: 20 - protein, 5 aa, synthetic construct
  source 1..5: note = linker sequence
GGGGS

SEQ ID NO: 21 - protein, 25 aa, synthetic construct
  source 1..25: note = linker sequence
GGGGSGGGGSGASAAGGGGSGGGGS

SEQ ID NO: 22 - protein, 25 aa, synthetic construct
  source 1..25: note = linker sequence
GGGGSGGGGSGGGGSGGGGSGGGGS

SEQ ID NO: 23 - protein, 44 aa, Homo sapiens
TTTPAPRPPTPAPTIASQPLSLRPEACRPAAGGAVHTRGLDFAC

SEQ ID NO: 24 - protein, 54 aa, Homo sapiens
FVPVFLPAKPTTTPAPRPPTPAPTIASQPLSLRPEACRPAAGGAVHTRGLDFAC

SEQ ID NO: 25 - protein, 39 aa, Homo sapiens
IEVMYPPPYLDNEKSNGTIIHVKGKHLCPSPLFPGPSKP

SEQ ID NO: 26 - protein, 133 aa, synthetic construct
  source 1..133: note = CD28 extracellular hinge domain
KILVKQSPMLVAYDNAVNLSCKYSYNLFSREFRASLHKGLDSAVEVCVVYGNYSQQLQVYSKTGFNCDGKLGNESVTFYLQNLYVNQTDIYFCKIEVMAPPPALDNEKSNGTIIHVKGKHLCPSPLFPGPSKP

SEQ ID NO: 27 - protein, 12 aa, synthetic construct
  source 1..12: note = IgG4 extracellular hinge domain
ESKYGPPCPPCP

SEQ ID NO: 28 - protein, 25 aa, Homo sapiens
DIYIWAPLAGTCGVLLLSLVITLYC

SEQ ID NO: 29 - protein, 28 aa, Homo sapiens
MFWVLVVVGGVLACYSLLVTVAFIIFWV

SEQ ID NO: 30 - protein, 69 aa, synthetic construct
  source 1..69: note = extracellular hinge und transmembrane domain
TTTPAPRPPTPAPTIASQPLSLRPEACRPAAGGAVHTRGLDFACDIYIWAPLAGTCGVLLLSLVITLYC

SEQ ID NO: 31 - protein, 83 aa, synthetic construct
  source 1..83: note = extracellular hinge und transmembrane domain
FVPVFLPAKPTTTPAPRPPTPAPTIASQPLSLRPEACRPAAGGAVHTRGLDFACDIYIWAPLAGTCGVLLLSLVITLYCNHRN

SEQ ID NO: 32 - protein, 66 aa, synthetic construct
  source 1..66: note = extracellular hinge und transmembrane domain
IEVMYPPPYLDNEKSNGTIIHVKGKHLCPSPLFPGPSKPFWVLVVVGGVLACYSLLVTVAFIIFWV

SEQ ID NO: 33 - protein, 37 aa, synthetic construct
  source 1..37: note = extracellular hinge und transmembrane domain
ESKYGPPCPPCPDIYIWAPLAGTCGVLLLSLVITLYC

SEQ ID NO: 34 - protein, 45 aa, synthetic construct
  source 1..45: note = extracellular hinge und transmembrane domain
ESKYGPPCPPCPTRGLDFACDIYIWAPLAGTCGVLLLSLVITLYC

SEQ ID NO: 35 - protein, 40 aa, synthetic construct
  source 1..40: note = extracellular hinge und transmembrane domain
ESKYGPPCPPCPMFWVLVVVGGVLACYSLLVTVAFIIFWV

SEQ ID NO: 36 - protein, 160 aa, synthetic construct
  source 1..160: note = extracellular hinge und transmembrane domain
KILVKQSPMLVAYDNAVNLSCKYSYNLFSREFRASLHKGLDSAVEVCVVYGNYSQQLQVYSKTGFNCDGKLGNESVTFYLQNLYVNQTDIYFCKIEVMAPPPALDNEKSNGTIIHVKGKHLCPSPLFPGPSKPFWVLVVVGGVLACYSLLVTVAFIIFWV

SEQ ID NO: 37 - protein, 41 aa, Homo sapiens
RSKRSRLLHSDYMNMTPRRPGPTRKHYQPYAPPRDFAAYRS

SEQ ID NO: 38 - protein, 41 aa, synthetic construct
  source 1..41: note = CD28 intracellular signaling domain
RSKRSRGGHSDYMNMTPRRPGPTRKHYQPYAPPRDFAAYRS

SEQ ID NO: 39 - protein, 42 aa, Homo sapiens
KRGRKKLLYIFKQPFMRPVQTTQEEDGCSCRFPEEEEGGCEL

SEQ ID NO: 40 - protein, 42 aa, synthetic construct
  source 1..42: note = 4-1BB intracellular signaling domain
KRGRKKGGYIFKQPFMRPVQTTQEEDGCSCRFPEEEEGGCEL

SEQ ID NO: 41 - protein, 112 aa, Homo sapiens
RVKFSRSADAPAYQQGQNQLYNELNLGRREEYDVLDKRRGRDPEMGGKPRRKNPQEGLYNELQKDKMAEAYSEIGMKGERRRGKGHDGLYQGLSTATKDTYDALHMQALPPR

SEQ ID NO: 42 - protein, 22 aa, Homo sapiens
MDMRVPAQLLGLLLLWLRGARC

SEQ ID NO: 43 - protein, 20 aa, synthetic construct
  source 1..20: note = leader peptide
MRRMQLLLLIALSLALVTNS

SEQ ID NO: 44 - protein, 21 aa, Homo sapiens
MKWKALFTAAILQAQLPITEA

SEQ ID NO: 45 - protein, 22 aa, Homo sapiens
MLLLVTSLLLCELPHPAFLLIP

SEQ ID NO: 46 - protein, 21 aa, Homo sapiens
MALPVTALLLPLALLLHAARP

SEQ ID NO: 47 - DNA, 66 bp, Homo sapiens
  source 1..66: mol_type = other DNA
atggacatgagagtgcccgctcaactgctgggactgctgctgctttggctgagaggcgccagatgc

SEQ ID NO: 48 - DNA, 60 bp, synthetic construct
  source 1..60: mol_type = other DNA; note = nucleic acid sequence encoding leader peptide
atgcggagaatgcagctgctgctgctcattgccctgtctctggccctggtcaccaacagc

SEQ ID NO: 49 - DNA, 63 bp, Homo sapiens
  source 1..63: mol_type = other DNA
atgaagtggaaggccctgttcacagccgccatcctgcaagcccagctgcctattacagaggcc

SEQ ID NO: 50 - DNA, 66 bp, Homo sapiens
  source 1..66: mol_type = other DNA
atgctgctgctggtcacaagcctgctgctgtgcgaactgccccatcctgcctttctgctgatcccc

SEQ ID NO: 51 - DNA, 63 bp, Homo sapiens
  source 1..63: mol_type = other DNA
atggctctgcctgtgacagctctgctgctgcctctggctctgcttctgcatgctgccagacct

SEQ ID NO: 52 - protein, 369 aa, synthetic construct
  source 1..369: note = switchable chimeric antigen receptor
MDMRVPAQLLGLLLLWLRGARCEFKPLPEVTDEYAAAGPGGGGSKILVKQSPMLVAYDNAVNLSCKYSYNLFSREFRASLHKGLDSAVEVCVVYGNYSQQLQVYSKTGFNCDGKLGNESVTFYLQNLYVNQTDIYFCKIEVMAPPPALDNEKSNGTIIHVKGKHLCPSPLFPGPSKPFWVLVVVGGVLACYSLLVTVAFIIFWVRSKRSRGGHSDYMNMTPRRPGPTRKHYQPYAPPRDFAAYRSGGGGSGGGASGGGGSFSRSADAPAYQQGQNQLYNELNLGRREEYDVLDKRRGRDPEMGGKPRRKNPQEGLYNELQKDKMAEAYSEIGMKGERRRGKGHDGLYQGLSTATKDTYGALHMQALPPR

SEQ ID NO: 53 - protein, 220 aa, synthetic construct
  source 1..220: note = switchable chimeric antigen receptor
EFKPLPEVTDEYAAAGGSGGSESKYGPPCPPCPTRGLDFACDIYIWAPLAGTCGVLLLSLVITLYCKRGRKKLLYIFKQPFMRPVQTTQEEDGCSCRFPEEEEGGCELRVKFSRSADAPAYKQGQNQLYNELNLGRREEYDVLDKRRGRDPEMGGKPRRKNPQEGLYNELQKDKMAEAYSEIGMKGERRRGKGHDGLYQGLSTATKDTYDALHMQALPPR

SEQ ID NO: 54 - protein, 244 aa, synthetic construct
  source 1..244: note = switchable chimeric antigen receptor
EFKPLPEVTDEYAAAGGSGGSTTTPAPRPPTPAPTIASQPLSLRPEACRPAAGGAVHTRGLDFACDIYIWAPLAGTCGVLLLSLVITLYCKRGRKKLLYIFKQPFMRPVQTTQEEDGCSCRFPEEEEGGCELRVKFSRSADAPAYKQGQNQLYNELNLGRREEYDVLDKRRGRDPEMGGKPRRKNPQEGLYNELQKDKMAEAYSEIGMKGERRRGKGHDGLYQGLSTATKDTYDALHMQALPPR

SEQ ID NO: 55 - protein, 240 aa, synthetic construct
  source 1..240: note = switchable chimeric antigen receptor
EFKPLPEVTDEYAAAGGSGGSIEVMYPPPYLDNEKSNGTIIHVKGKHLCPSPLFPGPSKPFWVLVVVGGVLACYSLLVTVAFIIFWVRSKRSRLLHSDYMNMTPRRPGPTRKHYQPYAPPRDFAAYRSRVKFSRSADAPAYQQGQNQLYNELNLGRREEYDVLDKRRGRDPEMGGKPRRKNPQEGLYNELQKDKMAEAYSEIGMKGERRRGKGHDGLYQGLSTATKDTYDALHMQALPPR

SEQ ID NO: 56 - protein, 257 aa, synthetic construct
  source 1..257: note = switchable chimeric antigen receptor
EFKPLPEVTDEYAAAGGSGGSFVPVFLPAKPTTTPAPRPPTPAPTIASQPLSLRPEACRPAAGGAVHTRGLDFACDIYIWAPLAGTCGVLLLSLVITLYCNHRNRSKRSRLLHSDYMNMTPRRPGPTRKHYQPYAPPRDFAAYRSRVKFSRSADAPAYQQGQNQLYNELNLGRREEYDVLDKRRGRDPEMGGKPRRKNPQEGLYNELQKDKMAEAYSEIGMKGERRRGKGHDGLYQGLSTATKDTYDALHMQALPPR

SEQ ID NO: 57 - protein, 239 aa, synthetic construct
  source 1..239: note = switchable chimeric antigen receptor
EFKPLPEVTDEYGGSGGSGGSKPLPEVTDEYAAAGGSGGSESKYGPPCPPCPTRGLDFACDIYIWAPLAGTCGVLLLSLVITLYCKRGRKKLLYIFKQPFMRPVQTTQEEDGCSCRFPEEEEGGCELRVKFSRSADAPAYKQGQNQLYNELNLGRREEYDVLDKRRGRDPEMGGKPRRKNPQEGLYNELQKDKMAEAYSEIGMKGERRRGKGHDGLYQGLSTATKDTYDALHMQALPPR

SEQ ID NO: 58 - protein, 258 aa, synthetic construct
  source 1..258: note = switchable chimeric antigen receptor
EFKPLPEVTDEYGGSGGSGGSKPLPEVTDEYGGSGGSGGSKPLPEVTDEYAAAGGSGGSESKYGPPCPPCPTRGLDFACDIYIWAPLAGTCGVLLLSLVITLYCKRGRKKLLYIFKQPFMRPVQTTQEEDGCSCRFPEEEEGGCELRVKFSRSADAPAYKQGQNQLYNELNLGRREEYDVLDKRRGRDPEMGGKPRRKNPQEGLYNELQKDKMAEAYSEIGMKGERRRGKGHDGLYQGLSTATKDTYDALHMQALPPR

SEQ ID NO: 59 - protein, 347 aa, synthetic construct
  source 1..347: note = switchable chimeric antigen receptor
EFKPLPEVTDEYAAAGPGGGGSKILVKQSPMLVAYDNAVNLSCKYSYNLFSREFRASLHKGLDSAVEVCVVYGNYSQQLQVYSKTGFNCDGKLGNESVTFYLQNLYVNQTDIYFCKIEVMAPPPALDNEKSNGTIIHVKGKHLCPSPLFPGPSKPFWVLVVVGGVLACYSLLVTVAFIIFWVRSRRSRGGHSDYMNMTPRRPGPTRKHYQPYAPPRDFAAYRSGGGGSGGGASGGGGSFSRSADAPAYQQGQNQLYNELNLGRREEYDVLDRRRGRDPEMGGRPRRRNPQEGLYNELQRDRMAEAYSEIGMRGERRRGRGHDGLYQGLSTATRDTYGALHMQALPPR

SEQ ID NO: 60 - protein, 349 aa, synthetic construct
  source 1..349: note = switchable chimeric antigen receptor
EFSKPLPEVTDEYKNAAAGGSGGSKILVKQSPMLVAYDNAVNLSCKYSYNLFSREFRASLHKGLDSAVEVCVVYGNYSQQLQVYSKTGFNCDGKLGNESVTFYLQNLYVNQTDIYFCKIEVMAPPPALDNEKSNGTIIHVKGKHLCPSPLFPGPSKPFWVLVVVGGVLACYSLLVTVAFIIFWVRSKRSRGGHSDYMNMTPRRPGPTRKHYQPYAPPRDFAAYRSGGGGSGGGASGGGGSFSRSADAPAYQQGQNQLYNELNLGRREEYDVLDKRRGRDPEMGGKPRRKNPQEGLYNELQKDKMAEAYSEIGMKGERRRGKGHDGLYQGLSTATKDTYGALHMQALPPR

SEQ ID NO: 61 - protein, 203 aa, synthetic construct
  source 1..203: note = switchable chimeric antigen receptor
EFKPLPEVTDEYESKYGPPCPPCPDIYIWAPLAGTCGVLLLSLVITLYCKRGRKKLLYIFKQPFMRPVQTTQEEDGCSCRFPEEEEGGCELRVKFSRSADAPAYQQGQNQLYNELNLGRREEYDVLDKRRGRDPEMGGKPRRKNPQEGLYNELQKDKMAEAYSEIGMKGERRRGKGHDGLYQGLSTATKDTYDALHMQALPPR

SEQ ID NO: 62 - protein, 206 aa, synthetic construct
  source 1..206: note = switchable chimeric antigen receptor
EFKPLPEVTDEYAAAESKYGPPCPPCPDIYIWAPLAGTCGVLLLSLVITLYCKRGRKKLLYIFKQPFMRPVQTTQEEDGCSCRFPEEEEGGCELRVKFSRSADAPAYQQGQNQLYNELNLGRREEYDVLDKRRGRDPEMGGKPRRKNPQEGLYNELQKDKMAEAYSEIGMKGERRRGKGHDGLYQGLSTATKDTYDALHMQALPPR

SEQ ID NO: 63 - protein, 212 aa, synthetic construct
  source 1..212: note = switchable chimeric antigen receptor
EFKPLPEVTDEYAAAGGSGGSESKYGPPCPPCPDIYIWAPLAGTCGVLLLSLVITLYCKRGRKKLLYIFKQPFMRPVQTTQEEDGCSCRFPEEEEGGCELRVKFSRSADAPAYQQGQNQLYNELNLGRREEYDVLDKRRGRDPEMGGKPRRKNPQEGLYNELQKDKMAEAYSEIGMKGERRRGKGHDGLYQGLSTATKDTYDALHMQALPPR

SEQ ID NO: 64 - protein, 207 aa, synthetic construct
  source 1..207: note = switchable chimeric antigen receptor
SKPLPEVTDEYKNAAAESKYGPPCPPCPDIYIWAPLAGTCGVLLLSLVITLYCKRGRKKLLYIFKQPFMRPVQTTQEEDGCSCRFPEEEEGGCELRVKFSRSADAPAYQQGQNQLYNELNLGRREEYDVLDKRRGRDPEMGGKPRRKNPQEGLYNELQKDKMAEAYSEIGMKGERRRGKGHDGLYQGLSTATKDTYDALHMQALPPR

SEQ ID NO: 65 - protein, 373 aa, synthetic construct
  source 1..373: note = switchable chimeric antigen receptor
ENGDNEKMAALEAKICHQIEYYFGDFNLPRDKFLKEQIKLDEGWVPLEIMIKFNRLNRLTTDFNVIVEALSKSKAELMEISEDKTKIRRSPSKPLPEVTDEYKNDVKNRSVYIKGFPTDATLDDIKEWLEDKGQVLNIQMRRTLHKAFKGSIFVVFDSIESAKKFVETPGQKYKETDLLILFESKYGPPCPPCPDIYIWAPLAGTCGVLLLSLVITLYCKRGRKKLLYIFKQPFMRPVQTTQEEDGCSCRFPEEEEGGCELRVKFSRSADAPAYQQGQNQLYNELNLGRREEYDVLDKRRGRDPEMGGKPRRKNPQEGLYNELQKDKMAEAYSEIGMKGERRRGKGHDGLYQGLSTATKDTYDALHMQALPPR

SEQ ID NO: 66 - protein, 220 aa, synthetic construct
  source 1..220: note = switchable chimeric antigen receptor
EFKPLPEVTDEYGGGGSEFKPLPEVTDEYESKYGPPCPPCPDIYIWAPLAGTCGVLLLSLVITLYCKRGRKKLLYIFKQPFMRPVQTTQEEDGCSCRFPEEEEGGCELRVKFSRSADAPAYQQGQNQLYNELNLGRREEYDVLDKRRGRDPEMGGKPRRKNPQEGLYNELQKDKMAEAYSEIGMKGERRRGKGHDGLYQGLSTATKDTYDALHMQALPPR

SEQ ID NO: 67 - protein, 208 aa, synthetic construct
  source 1..208: note = switchable chimeric antigen receptor
EFKPLPEVTDEYAAAESKYGPPCPPCPMFWVLVVVGGVLACYSLLVTVAFIIFWVRSKRSRLLHSDYMNMTPRRPGPTRKHYQPYAPPRDFAAYRSRVKFSRSADAPAYQQGQNQLYNELNLGRREEYDVLDKRRGRDPEMGGKPRRKNPQEGLYNELQKDKMAEAYSEIGMKGERRRGKGHDGLYQGLSTATKDTYDALHMQALPPR

SEQ ID NO: 68 - protein, 209 aa, synthetic construct
  source 1..209: note = switchable chimeric antigen receptor
EFKPLPEVTDEYAAAESKYGPPCPPCPMFWVLVVVGGVLACYSLLVTVAFIIFWVKRGRKKLLYIFKQPFMRPVQTTQEEDGCSCRFPEEEEGGCELRVKFSRSADAPAYQQGQNQLYNELNLGRREEYDVLDKRRGRDPEMGGKPRRKNPQEGLYNELQKDKMAEAYSEIGMKGERRRGKGHDGLYQGLSTATKDTYDALHMQALPPR

SEQ ID NO: 69 - protein, 222 aa, synthetic construct
  source 1..222: note = switchable chimeric antigen receptor
EFKPLPEVTDEYGGGGSEFKPLPEVTDEYESKYGPPCPPCPMFWVLVVVGGVLACYSLLVTVAFIIFWVRSKRSRLLHSDYMNMTPRRPGPTRKHYQPYAPPRDFAAYRSRVKFSRSADAPAYQQGQNQLYNELNLGRREEYDVLDKRRGRDPEMGGKPRRKNPQEGLYNELQKDKMAEAYSEIGMKGERRRGKGHDGLYQGLSTATKDTYDALHMQALPPR

SEQ ID NO: 70 - protein, 222 aa, synthetic construct
  source 1..222: note = switchable chimeric antigen receptor
EFKPLPEVTDEYGGGGSEFKPLPEVTDEYESKYGPPCPPCPMFWVLVVVGGVLACYSLLVTVAFIIFWVRSKRSRGGHSDYMNMTPRRPGPTRKHYQPYAPPRDFAAYRSRVKFSRSADAPAYQQGQNQLYNELNLGRREEYDVLDKRRGRDPEMGGKPRRKNPQEGLYNELQKDKMAEAYSEIGMKGERRRGKGHDGLYQGLSTATKDTYDALHMQALPPR

SEQ ID NO: 71 - protein, 219 aa, synthetic construct
  source 1..219: note = switchable chimeric antigen receptor
EFKPLPEVTDEYGGGGSEFKPLPEVTDEYESKYGPPCPPCPDIYIWAPLAGTCGVLLLSLVITLYCRSKRSRGGHSDYMNMTPRRPGPTRKHYQPYAPPRDFAAYRSRVKFSRSADAPAYQQGQNQLYNELNLGRREEYDVLDKRRGRDPEMGGKPRRKNPQEGLYNELQKDKMAEAYSEIGMKGERRRGKGHDGLYQGLSTATKDTYDALHMQALPPR

SEQ ID NO: 72 - protein, 223 aa, synthetic construct
  source 1..223: note = switchable chimeric antigen receptor
EFKPLPEVTDEYGGGGSEFKPLPEVTDEYESKYGPPCPPCPMFWVLVVVGGVLACYSLLVTVAFIIFWVKRGRKKLLYIFKQPFMRPVQTTQEEDGCSCRFPEEEEGGCELRVKFSRSADAPAYQQGQNQLYNELNLGRREEYDVLDKRRGRDPEMGGKPRRKNPQEGLYNELQKDKMAEAYSEIGMKGERRRGKGHDGLYQGLSTATKDTYDALHMQALPPR

SEQ ID NO: 73 - protein, 223 aa, synthetic construct
  source 1..223: note = switchable chimeric antigen receptor
EFKPLPEVTDEYGGGGSEFKPLPEVTDEYESKYGPPCPPCPMFWVLVVVGGVLACYSLLVTVAFIIFWVKRGRKKGGYIFKQPFMRPVQTTQEEDGCSCRFPEEEEGGCELRVKFSRSADAPAYQQGQNQLYNELNLGRREEYDVLDKRRGRDPEMGGKPRRKNPQEGLYNELQKDKMAEAYSEIGMKGERRRGKGHDGLYQGLSTATKDTYDALHMQALPPR

SEQ ID NO: 74 - protein, 214 aa, synthetic construct
  source 1..214: note = switchable chimeric antigen receptor
EFKPLPEVTDEYAAAGGSGGSESKYGPPCPPCPMFWVLVVVGGVLACYSLLVTVAFIIFWVRSKRSRLLHSDYMNMTPRRPGPTRKHYQPYAPPRDFAAYRSRVKFSRSADAPAYQQGQNQLYNELNLGRREEYDVLDKRRGRDPEMGGKPRRKNPQEGLYNELQKDKMAEAYSEIGMKGERRRGKGHDGLYQGLSTATKDTYDALHMQALPPR

SEQ ID NO: 75 - protein, 214 aa, synthetic construct
  source 1..214: note = switchable chimeric antigen receptor
EFKPLPEVTDEYAAAGGSGGSESKYGPPCPPCPMFWVLVVVGGVLACYSLLVTVAFIIFWVRSKRSRGGHSDYMNMTPRRPGPTRKHYQPYAPPRDFAAYRSRVKFSRSADAPAYQQGQNQLYNELNLGRREEYDVLDKRRGRDPEMGGKPRRKNPQEGLYNELQKDKMAEAYSEIGMKGERRRGKGHDGLYQGLSTATKDTYDALHMQALPPR

SEQ ID NO: 76 - protein, 211 aa, synthetic construct
  source 1..211: note = switchable chimeric antigen receptor
EFKPLPEVTDEYAAAGGSGGSESKYGPPCPPCPDIYIWAPLAGTCGVLLLSLVITLYCRSKRSRGGHSDYMNMTPRRPGPTRKHYQPYAPPRDFAAYRSRVKFSRSADAPAYQQGQNQLYNELNLGRREEYDVLDKRRGRDPEMGGKPRRKNPQEGLYNELQKDKMAEAYSEIGMKGERRRGKGHDGLYQGLSTATKDTYDALHMQALPPR

SEQ ID NO: 77 - protein, 215 aa, synthetic construct
  source 1..215: note = switchable chimeric antigen receptor
EFKPLPEVTDEYAAAGGSGGSESKYGPPCPPCPMFWVLVVVGGVLACYSLLVTVAFIIFWVKRGRKKLLYIFKQPFMRPVQTTQEEDGCSCRFPEEEEGGCELRVKFSRSADAPAYQQGQNQLYNELNLGRREEYDVLDKRRGRDPEMGGKPRRKNPQEGLYNELQKDKMAEAYSEIGMKGERRRGKGHDGLYQGLSTATKDTYDALHMQALPPR

SEQ ID NO: 78 - protein, 215 aa, synthetic construct
  source 1..215: note = switchable chimeric antigen receptor
EFKPLPEVTDEYAAAGGSGGSESKYGPPCPPCPMFWVLVVVGGVLACYSLLVTVAFIIFWVKRGRKKGGYIFKQPFMRPVQTTQEEDGCSCRFPEEEEGGCELRVKFSRSADAPAYQQGQNQLYNELNLGRREEYDVLDKRRGRDPEMGGKPRRKNPQEGLYNELQKDKMAEAYSEIGMKGERRRGKGHDGLYQGLSTATKDTYDALHMQALPPR

SEQ ID NO: 79 - protein, 246 aa, synthetic construct
  source 1..246: note = switchable chimeric antigen receptor
EFKPLPEVTDEYGGGGSEFKPLPEVTDEYIEVMYPPPYLDNEKSNGTIIHVKGKHLCPSPLFPGPSKPDIYIWAPLAGTCGVLLLSLVITLYCRSKRSRGGHSDYMNMTPRRPGPTRKHYQPYAPPRDFAAYRSRVKFSRSADAPAYQQGQNQLYNELNLGRREEYDVLDKRRGRDPEMGGKPRRKNPQEGLYNELQKDKMAEAYSEIGMKGERRRGKGHDGLYQGLSTATKDTYDALHMQALPPR

SEQ ID NO: 80 - protein, 205 aa, synthetic construct
  source 1..205: note = switchable chimeric antigen receptor
EFKPLPEVTDEYESKYGPPCPPCPMFWVLVVVGGVLACYSLLVTVAFIIFWVRSKRSRGGHSDYMNMTPRRPGPTRKHYQPYAPPRDFAAYRSRVKFSRSADAPAYQQGQNQLYNELNLGRREEYDVLDKRRGRDPEMGGKPRRKNPQEGLYNELQKDKMAEAYSEIGMKGERRRGKGHDGLYQGLSTATKDTYDALHMQALPPR

SEQ ID NO: 81 - protein, 206 aa, synthetic construct
  source 1..206: note = switchable chimeric antigen receptor
EFKPLPEVTDEYESKYGPPCPPCPMFWVLVVVGGVLACYSLLVTVAFIIFWVKRGRKKGGYIFKQPFMRPVQTTQEEDGCSCRFPEEEEGGCELRVKFSRSADAPAYQQGQNQLYNELNLGRREEYDVLDKRRGRDPEMGGKPRRKNPQEGLYNELQKDKMAEAYSEIGMKGERRRGKGHDGLYQGLSTATKDTYDALHMQALPPR

SEQ ID NO: 82 - protein, 212 aa, synthetic construct; identical to SEQ ID NO: 63
  source 1..212: note = switchable chimeric antigen receptor

SEQ ID NO: 83 - protein, 242 aa, synthetic construct
  source 1..242: note = switchable chimeric antigen receptor
MDMRVPAQLLGLLLLWLRGARCEFKPLPEVTDEYAAAGGSGGSESKYGPPCPPCPTRGLDFACDIYIWAPLAGTCGVLLLSLVITLYCKRGRKKLLYIFKQPFMRPVQTTQEEDGCSCRFPEEEEGGCELRVKFSRSADAPAYKQGQNQLYNELNLGRREEYDVLDKRRGRDPEMGGKPRRKNPQEGLYNELQKDKMAEAYSEIGMKGERRRGKGHDGLYQGLSTATKDTYDALHMQALPPR

SEQ ID NO: 84 - protein, 266 aa, synthetic construct
  source 1..266: note = switchable chimeric antigen receptor
MDMRVPAQLLGLLLLWLRGARCEFKPLPEVTDEYAAAGGSGGSTTTPAPRPPTPAPTIASQPLSLRPEACRPAAGGAVHTRGLDFACDIYIWAPLAGTCGVLLLSLVITLYCKRGRKKLLYIFKQPFMRPVQTTQEEDGCSCRFPEEEEGGCELRVKFSRSADAPAYKQGQNQLYNELNLGRREEYDVLDKRRGRDPEMGGKPRRKNPQEGLYNELQKDKMAEAYSEIGMKGERRRGKGHDGLYQGLSTATKDTYDALHMQALPPR

SEQ ID NO: 85 - protein, 262 aa, synthetic construct
  source 1..262: note = switchable chimeric antigen receptor
MDMRVPAQLLGLLLLWLRGARCEFKPLPEVTDEYAAAGGSGGSIEVMYPPPYLDNEKSNGTIIHVKGKHLCPSPLFPGPSKPFWVLVVVGGVLACYSLLVTVAFIIFWVRSKRSRLLHSDYMNMTPRRPGPTRKHYQPYAPPRDFAAYRSRVKFSRSADAPAYQQGQNQLYNELNLGRREEYDVLDKRRGRDPEMGGKPRRKNPQEGLYNELQKDKMAEAYSEIGMKGERRRGKGHDGLYQGLSTATKDTYDALHMQALPPR

SEQ ID NO: 86 - protein, 279 aa, synthetic construct
  source 1..279: note = switchable chimeric antigen receptor
MDMRVPAQLLGLLLLWLRGARCEFKPLPEVTDEYAAAGGSGGSFVPVFLPAKPTTTPAPRPPTPAPTIASQPLSLRPEACRPAAGGAVHTRGLDFACDIYIWAPLAGTCGVLLLSLVITLYCNHRNRSKRSRLLHSDYMNMTPRRPGPTRKHYQPYAPPRDFAAYRSRVKFSRSADAPAYQQGQNQLYNELNLGRREEYDVLDKRRGRDPEMGGKPRRKNPQEGLYNELQKDKMAEAYSEIGMKGERRRGKGHDGLYQGLSTATKDTYDALHMQALPPR

SEQ ID NO: 87 - protein, 261 aa, synthetic construct
  source 1..261: note = switchable chimeric antigen receptor
MDMRVPAQLLGLLLLWLRGARCEFKPLPEVTDEYGGSGGSGGSKPLPEVTDEYAAAGGSGGSESKYGPPCPPCPTRGLDFACDIYIWAPLAGTCGVLLLSLVITLYCKRGRKKLLYIFKQPFMRPVQTTQEEDGCSCRFPEEEEGGCELRVKFSRSADAPAYKQGQNQLYNELNLGRREEYDVLDKRRGRDPEMGGKPRRKNPQEGLYNELQKDKMAEAYSEIGMKGERRRGKGHDGLYQGLSTATKDTYDALHMQALPPR

SEQ ID NO: 88 - protein, 280 aa, synthetic construct
  source 1..280: note = switchable chimeric antigen receptor
MDMRVPAQLLGLLLLWLRGARCEFKPLPEVTDEYGGSGGSGGSKPLPEVTDEYGGSGGSGGSKPLPEVTDEYAAAGGSGGSESKYGPPCPPCPTRGLDFACDIYIWAPLAGTCGVLLLSLVITLYCKRGRKKLLYIFKQPFMRPVQTTQEEDGCSCRFPEEEEGGCELRVKFSRSADAPAYKQGQNQLYNELNLGRREEYDVLDKRRGRDPEMGGKPRRKNPQEGLYNELQKDKMAEAYSEIGMKGERRRGKGHDGLYQGLSTATKDTYDALHMQALPPR

SEQ ID NO: 89 - protein, 369 aa, synthetic construct
  source 1..369: note = switchable chimeric antigen receptor
MDMRVPAQLLGLLLLWLRGARCEFKPLPEVTDEYAAAGPGGGGSKILVKQSPMLVAYDNAVNLSCKYSYNLFSREFRASLHKGLDSAVEVCVVYGNYSQQLQVYSKTGFNCDGKLGNESVTFYLQNLYVNQTDIYFCKIEVMAPPPALDNEKSNGTIIHVKGKHLCPSPLFPGPSKPFWVLVVVGGVLACYSLLVTVAFIIFWVRSRRSRGGHSDYMNMTPRRPGPTRKHYQPYAPPRDFAAYRSGGGGSGGGASGGGGSFSRSADAPAYQQGQNQLYNELNLGRREEYDVLDRRRGRDPEMGGRPRRRNPQEGLYNELQRDRMAEAYSEIGMRGERRRGRGHDGLYQGLSTATRDTYGALHMQALPPR

SEQ ID NO: 90 - protein, 371 aa, synthetic construct
  source 1..371: note = switchable chimeric antigen receptor
MDMRVPAQLLGLLLLWLRGARCEFSKPLPEVTDEYKNAAAGGSGGSKILVKQSPMLVAYDNAVNLSCKYSYNLFSREFRASLHKGLDSAVEVCVVYGNYSQQLQVYSKTGFNCDGKLGNESVTFYLQNLYVNQTDIYFCKIEVMAPPPALDNEKSNGTIIHVKGKHLCPSPLFPGPSKPFWVLVVVGGVLACYSLLVTVAFIIFWVRSKRSRGGHSDYMNMTPRRPGPTRKHYQPYAPPRDFAAYRSGGGGSGGGASGGGGSFSRSADAPAYQQGQNQLYNELNLGRREEYDVLDKRRGRDPEMGGKPRRKNPQEGLYNELQKDKMAEAYSEIGMKGERRRGKGHDGLYQGLSTATKDTYGALHMQALPPR

SEQ ID NO: 91 - protein, 225 aa, synthetic construct
  source 1..225: note = switchable chimeric antigen receptor
MDMRVPAQLLGLLLLWLRGARCEFKPLPEVTDEYESKYGPPCPPCPDIYIWAPLAGTCGVLLLSLVITLYCKRGRKKLLYIFKQPFMRPVQTTQEEDGCSCRFPEEEEGGCELRVKFSRSADAPAYQQGQNQLYNELNLGRREEYDVLDKRRGRDPEMGGKPRRKNPQEGLYNELQKDKMAEAYSEIGMKGERRRGKGHDGLYQGLSTATKDTYDALHMQALPPR

SEQ ID NO: 92 - protein, 228 aa, synthetic construct
  source 1..228: note = switchable chimeric antigen receptor
MDMRVPAQLLGLLLLWLRGARCEFKPLPEVTDEYAAAESKYGPPCPPCPDIYIWAPLAGTCGVLLLSLVITLYCKRGRKKLLYIFKQPFMRPVQTTQEEDGCSCRFPEEEEGGCELRVKFSRSADAPAYQQGQNQLYNELNLGRREEYDVLDKRRGRDPEMGGKPRRKNPQEGLYNELQKDKMAEAYSEIGMKGERRRGKGHDGLYQGLSTATKDTYDALHMQALPPR

SEQ ID NO: 93 - protein, 234 aa, synthetic construct
  source 1..234: note = switchable chimeric antigen receptor
MDMRVPAQLLGLLLLWLRGARCEFKPLPEVTDEYAAAGGSGGSESKYGPPCPPCPDIYIWAPLAGTCGVLLLSLVITLYCKRGRKKLLYIFKQPFMRPVQTTQEEDGCSCRFPEEEEGGCELRVKFSRSADAPAYQQGQNQLYNELNLGRREEYDVLDKRRGRDPEMGGKPRRKNPQEGLYNELQKDKMAEAYSEIGMKGERRRGKGHDGLYQGLSTATKDTYDALHMQALPPR

SEQ ID NO: 94 - protein, 229 aa, synthetic construct
  source 1..229: note = switchable chimeric antigen receptor
MDMRVPAQLLGLLLLWLRGARCSKPLPEVTDEYKNAAAESKYGPPCPPCPDIYIWAPLAGTCGVLLLSLVITLYCKRGRKKLLYIFKQPFMRPVQTTQEEDGCSCRFPEEEEGGCELRVKFSRSADAPAYQQGQNQLYNELNLGRREEYDVLDKRRGRDPEMGGKPRRKNPQEGLYNELQKDKMAEAYSEIGMKGERRRGKGHDGLYQGLSTATKDTYDALHMQALPPR

SEQ ID NO: 95 - protein, 395 aa, synthetic construct
  source 1..395: note = switchable chimeric antigen receptor
MDMRVPAQLLGLLLLWLRGARCENGDNEKMAALEAKICHQIEYYFGDFNLPRDKFLKEQIKLDEGWVPLEIMIKFNRLNRLTTDFNVIVEALSKSKAELMEISEDKTKIRRSPSKPLPEVTDEYKNDVKNRSVYIKGFPTDATLDDIKEWLEDKGQVLNIQMRRTLHKAFKGSIFVVFDSIESAKKFVETPGQKYKETDLLILFESKYGPPCPPCPDIYIWAPLAGTCGVLLLSLVITLYCKRGRKKLLYIFKQPFMRPVQTTQEEDGCSCRFPEEEEGGCELRVKFSRSADAPAYQQGQNQLYNELNLGRREEYDVLDKRRGRDPEMGGKPRRKNPQEGLYNELQKDKMAEAYSEIGMKGERRRGKGHDGLYQGLSTATKDTYDALHMQALPPR

SEQ ID NO: 96 - protein, 242 aa, synthetic construct
  source 1..242: note = switchable chimeric antigen receptor
MDMRVPAQLLGLLLLWLRGARCEFKPLPEVTDEYGGGGSEFKPLPEVTDEYESKYGPPCPPCPDIYIWAPLAGTCGVLLLSLVITLYCKRGRKKLLYIFKQPFMRPVQTTQEEDGCSCRFPEEEEGGCELRVKFSRSADAPAYQQGQNQLYNELNLGRREEYDVLDKRRGRDPEMGGKPRRKNPQEGLYNELQKDKMAEAYSEIGMKGERRRGKGHDGLYQGLSTATKDTYDALHMQALPPR

SEQ ID NO: 97 - protein, 230 aa, synthetic construct
  source 1..230: note = switchable chimeric antigen receptor
MDMRVPAQLLGLLLLWLRGARCEFKPLPEVTDEYAAAESKYGPPCPPCPMFWVLVVVGGVLACYSLLVTVAFIIFWVRSKRSRLLHSDYMNMTPRRPGPTRKHYQPYAPPRDFAAYRSRVKFSRSADAPAYQQGQNQLYNELNLGRREEYDVLDKRRGRDPEMGGKPRRKNPQEGLYNELQKDKMAEAYSEIGMKGERRRGKGHDGLYQGLSTATKDTYDALHMQALPPR

SEQ ID NO: 98 - protein, 231 aa, synthetic construct
  source 1..231: note = switchable chimeric antigen receptor
MDMRVPAQLLGLLLLWLRGARCEFKPLPEVTDEYAAAESKYGPPCPPCPMFWVLVVVGGVLACYSLLVTVAFIIFWVKRGRKKLLYIFKQPFMRPVQTTQEEDGCSCRFPEEEEGGCELRVKFSRSADAPAYQQGQNQLYNELNLGRREEYDVLDKRRGRDPEMGGKPRRKNPQEGLYNELQKDKMAEAYSEIGMKGERRRGKGHDGLYQGLSTATKDTYDALHMQALPPR

SEQ ID NO: 99 - protein, 244 aa, synthetic construct
  source 1..244: note = switchable chimeric antigen receptor
MDMRVPAQLLGLLLLWLRGARCEFKPLPEVTDEYGGGGSEFKPLPEVTDEYESKYGPPCPPCPMFWVLVVVGGVLACYSLLVTVAFIIFWVRSKRSRLLHSDYMNMTPRRPGPTRKHYQPYAPPRDFAAYRSRVKFSRSADAPAYQQGQNQLYNELNLGRREEYDVLDKRRGRDPEMGGKPRRKNPQEGLYNELQKDKMAEAYSEIGMKGERRRGKGHDGLYQGLSTATKDTYDALHMQALPPR

SEQ ID NO: 100 - protein, 244 aa, synthetic construct
  source 1..244: note = switchable chimeric antigen receptor
MDMRVPAQLLGLLLLWLRGARCEFKPLPEVTDEYGGGGSEFKPLPEVTDEYESKYGPPCPPCPMFWVLVVVGGVLACYSLLVTVAFIIFWVRSKRSRGGHSDYMNMTPRRPGPTRKHYQPYAPPRDFAAYRSRVKFSRSADAPAYQQGQNQLYNELNLGRREEYDVLDKRRGRDPEMGGKPRRKNPQEGLYNELQKDKMAEAYSEIGMKGERRRGKGHDGLYQGLSTATKDTYDALHMQALPPR

SEQ ID NO: 101 - protein, 241 aa, synthetic construct
  source 1..241: note = switchable chimeric antigen receptor
MDMRVPAQLLGLLLLWLRGARCEFKPLPEVTDEYGGGGSEFKPLPEVTDEYESKYGPPCPPCPDIYIWAPLAGTCGVLLLSLVITLYCRSKRSRGGHSDYMNMTPRRPGPTRKHYQPYAPPRDFAAYRSRVKFSRSADAPAYQQGQNQLYNELNLGRREEYDVLDKRRGRDPEMGGKPRRKNPQEGLYNELQKDKMAEAYSEIGMKGERRRGKGHDGLYQGLSTATKDTYDALHMQALPPR

SEQ ID NO: 102 - protein, 245 aa, synthetic construct
  source 1..245: note = switchable chimeric antigen receptor
MDMRVPAQLLGLLLLWLRGARCEFKPLPEVTDEYGGGGSEFKPLPEVTDEYESKYGPPCPPCPMFWVLVVVGGVLACYSLLVTVAFIIFWVKRGRKKLLYIFKQPFMRPVQTTQEEDGCSCRFPEEEEGGCELRVKFSRSADAPAYQQGQNQLYNELNLGRREEYDVLDKRRGRDPEMGGKPRRKNPQEGLYNELQKDKMAEAYSEIGMKGERRRGKGHDGLYQGLSTATKDTYDALHMQALPPR

SEQ ID NO: 103 - protein, 245 aa, synthetic construct
  source 1..245: note = switchable chimeric antigen receptor
MDMRVPAQLLGLLLLWLRGARCEFKPLPEVTDEYGGGGSEFKPLPEVTDEYESKYGPPCPPCPMFWVLVVVGGVLACYSLLVTVAFIIFWVKRGRKKGGYIFKQPFMRPVQTTQEEDGCSCRFPEEEEGGCELRVKFSRSADAPAYQQGQNQLYNELNLGRREEYDVLDKRRGRDPEMGGKPRRKNPQEGLYNELQKDKMAEAYSEIGMKGERRRGKGHDGLYQGLSTATKDTYDALHMQALPPR

SEQ ID NO: 104 - protein, 236 aa, synthetic construct
  source 1..236: note = switchable chimeric antigen receptor
MDMRVPAQLLGLLLLWLRGARCEFKPLPEVTDEYAAAGGSGGSESKYGPPCPPCPMFWVLVVVGGVLACYSLLVTVAFIIFWVRSKRSRLLHSDYMNMTPRRPGPTRKHYQPYAPPRDFAAYRSRVKFSRSADAPAYQQGQNQLYNELNLGRREEYDVLDKRRGRDPEMGGKPRRKNPQEGLYNELQKDKMAEAYSEIGMKGERRRGKGHDGLYQGLSTATKDTYDALHMQALPPR

SEQ ID NO: 105 - protein, 236 aa, synthetic construct
  source 1..236: note = switchable chimeric antigen receptor
MDMRVPAQLLGLLLLWLRGARCEFKPLPEVTDEYAAAGGSGGSESKYGPPCPPCPMFWVLVVVGGVLACYSLLVTVAFIIFWVRSKRSRGGHSDYMNMTPRRPGPTRKHYQPYAPPRDFAAYRSRVKFSRSADAPAYQQGQNQLYNELNLGRREEYDVLDKRRGRDPEMGGKPRRKNPQEGLYNELQKDKMAEAYSEIGMKGERRRGKGHDGLYQGLSTATKDTYDALHMQALPPR

SEQ ID NO: 106 - protein, 233 aa, synthetic construct
  source 1..233: note = switchable chimeric antigen receptor
MDMRVPAQLLGLLLLWLRGARCEFKPLPEVTDEYAAAGGSGGSESKYGPPCPPCPDIYIWAPLAGTCGVLLLSLVITLYCRSKRSRGGHSDYMNMTPRRPGPTRKHYQPYAPPRDFAAYRSRVKFSRSADAPAYQQGQNQLYNELNLGRREEYDVLDKRRGRDPEMGGKPRRKNPQEGLYNELQKDKMAEAYSEIGMKGERRRGKGHDGLYQGLSTATKDTYDALHMQALPPR

SEQ ID NO: 107 - protein, 237 aa, synthetic construct
  source 1..237: note = switchable chimeric antigen receptor
MDMRVPAQLLGLLLLWLRGARCEFKPLPEVTDEYAAAGGSGGSESKYGPPCPPCPMFWVLVVVGGVLACYSLLVTVAFIIFWVKRGRKKLLYIFKQPFMRPVQTTQEEDGCSCRFPEEEEGGCELRVKFSRSADAPAYQQGQNQLYNELNLGRREEYDVLDKRRGRDPEMGGKPRRKNPQEGLYNELQKDKMAEAYSEIGMKGERRRGKGHDGLYQGLSTATKDTYDALHMQALPPR

SEQ ID NO: 108 - protein, 237 aa, synthetic construct
  source 1..237: note = switchable chimeric antigen receptor
MDMRVPAQLLGLLLLWLRGARCEFKPLPEVTDEYAAAGGSGGSESKYGPPCPPCPMFWVLVVVGGVLACYSLLVTVAFIIFWVKRGRKKGGYIFKQPFMRPVQTTQEEDGCSCRFPEEEEGGCELRVKFSRSADAPAYQQGQNQLYNELNLGRREEYDVLDKRRGRDPEMGGKPRRKNPQEGLYNELQKDKMAEAYSEIGMKGERRRGKGHDGLYQGLSTATKDTYDALHMQALPPR

SEQ ID NO: 109 - protein, 268 aa, synthetic construct
  source 1..268: note = switchable chimeric antigen receptor
MDMRVPAQLLGLLLLWLRGARCEFKPLPEVTDEYGGGGSEFKPLPEVTDEYIEVMYPPPYLDNEKSNGTIIHVKGKHLCPSPLFPGPSKPDIYIWAPLAGTCGVLLLSLVITLYCRSKRSRGGHSDYMNMTPRRPGPTRKHYQPYAPPRDFAAYRSRVKFSRSADAPAYQQGQNQLYNELNLGRREEYDVLDKRRGRDPEMGGKPRRKNPQEGLYNELQKDKMAEAYSEIGMKGERRRGKGHDGLYQGLSTATKDTYDALHMQALPPR

SEQ ID NO: 110 - protein, 227 aa, synthetic construct
  source 1..227: note = switchable chimeric antigen receptor
MDMRVPAQLLGLLLLWLRGARCEFKPLPEVTDEYESKYGPPCPPCPMFWVLVVVGGVLACYSLLVTVAFIIFWVRSKRSRGGHSDYMNMTPRRPGPTRKHYQPYAPPRDFAAYRSRVKFSRSADAPAYQQGQNQLYNELNLGRREEYDVLDKRRGRDPEMGGKPRRKNPQEGLYNELQKDKMAEAYSEIGMKGERRRGKGHDGLYQGLSTATKDTYDALHMQALPPR

SEQ ID NO: 111 - protein, 228 aa, synthetic construct
  source 1..228: note = switchable chimeric antigen receptor
MDMRVPAQLLGLLLLWLRGARCEFKPLPEVTDEYESKYGPPCPPCPMFWVLVVVGGVLACYSLLVTVAFIIFWVKRGRKKGGYIFKQPFMRPVQTTQEEDGCSCRFPEEEEGGCELRVKFSRSADAPAYQQGQNQLYNELNLGRREEYDVLDKRRGRDPEMGGKPRRKNPQEGLYNELQKDKMAEAYSEIGMKGERRRGKGHDGLYQGLSTATKDTYDALHMQALPPR

SEQ ID NO: 112 - protein, 234 aa, synthetic construct; identical to SEQ ID NO: 93
  source 1..234: note = switchable chimeric antigen receptor

SEQ ID NO: 113 - DNA, 660 bp, synthetic construct
  source 1..660: mol_type = other DNA; note = nucleic acid encoding switchable chimeric antigen receptor
gagttcaagcctctgcctgaagtgaccgatgagtatgccgctgctggtggatctggcggcagcgagtctaagtacggacctccttgtcctccatgtcctaccagaggcctggacttcgcctgcgacatctatatctgggcccctctggctggcacatgtggcgttttgctgctgagcctggtcatcaccctgtactgcaagcggggcagaaagaagctgctgtacatcttcaagcagcccttcatgcggcccgtgcagaccacacaagaggaagatggctgctcctgcagattccccgaggaagaagaaggcggctgcgagctgagagtgaagttcagcagatccgccgacgctcccgcctataagcagggacagaaccagctgtacaacgagctgaacctggggagaagagaagagtacgacgtgctggacaagcggagaggcagagatcctgagatgggcggcaagcccagacggaagaatcctcaagagggcctgtataatgagctgcagaaagacaagatggccgaggcctacagcgagatcggaatgaagggcgagcgcagaagaggcaagggacacgatggactgtaccagggcctgagcaccgccaccaaggatacctatgatgccctgcacatgcaggccctgcctccaaga

SEQ ID NO: 114 - DNA, 732 bp, synthetic construct
  source 1..732: mol_type = other DNA; note = nucleic acid encoding switchable chimeric antigen receptor
gagttcaagcctctgcctgaagtgaccgatgagtatgccgctgctggtggatctggcggcagcacaacaacaccagctcctagaccacctacaccagcacctaccattgccagccagcctctgtctctgaggccagaggcatgtagacctgctgctggcggagccgtgcatacaagaggactggatttcgcctgcgacatctacatctgggcccctctggctggaacatgtggcgttctgctgctgagcctggtcatcaccctgtactgcaagcggggcagaaagaagctgctgtacatcttcaagcagcccttcatgcggcccgtgcagaccacacaagaggaagatggctgctcctgcagattccccgaggaagaagaaggcggctgcgagctgagagtgaagttcagcagatccgccgacgctcccgcctataagcagggacagaaccagctgtacaacgagctgaacctggggagaagagaagagtacgacgtgctggacaagcggagaggcagagatcctgagatgggcggcaagcccagacggaagaatcctcaagagggcctgtataatgagctgcagaaagacaagatggccgaggcctacagcgagatcggaatgaagggcgagcgcagaagaggcaagggacacgatggactgtaccagggcctgagcaccgccaccaaggatacctatgatgccctgcacatgcaggccctgcctccaaga

SEQ ID NO: 115 - DNA, 720 bp, synthetic construct
  source 1..720: mol_type = other DNA; note = nucleic acid encoding switchable chimeric antigen receptor
gagttcaagcctctgcctgaagtgaccgatgagtatgccgctgctggtggatctggcggcagcatcgaagtgatgtaccctccaccttacctggacaacgagaagtccaacggcaccatcatccacgtgaagggcaagcacctgtgtccttctccactgttccccggacctagcaagcctttctgggtgctcgttgttgttggcggcgtgctggcctgttacagcctgctggttaccgtggccttcatcatcttttgggtccgaagcaagcggagccggctgctgcacagcgactacatgaacatgacccctagacggcccggaccaaccagaaagcactaccagccttacgctcctcctagagacttcgccgcctaccggtccagagtgaagttcagcagatccgccgatgctcccgcctatcagcagggacagaaccagctgtacaacgagctgaacctggggagaagagaagagtacgacgtgctggacaagcggagaggcagagatcctgagatgggcggcaagcccagacggaagaatcctcaagagggcctgtataatgagctgcagaaagacaagatggccgaggcctacagcgagatcggaatgaagggcgagcgcagaagaggcaagggacacgatggactgtaccagggactgagcaccgccaccaaggatacctatgacgccctgcacatgcaggccctgcctccaaga

SEQ ID NO: 116 - DNA, 771 bp, synthetic construct
  source 1..771: mol_type = other DNA; note = nucleic acid encoding switchable chimeric antigen receptor
gagttcaagcctctgcctgaagtgaccgatgagtatgccgctgctggtggaagcggcggctctttcgttcctgtgttcctgcctgccaagcctaccaccacaccagctcctagacctccaactcctgctcctaccattgccagccagcctctgtctctgaggccagaggcatgtagacctgctgctggcggagccgtgcatacaagaggactggatttcgcctgcgacatctacatctgggcccctctggctggaacatgtggcgttctgctgctgagcctggtcatcaccctgtactgcaaccaccggaacagaagcaagcggagcagactgctgcacagcgactacatgaacatgacccctagacggcccggacctaccagaaagcactaccagccttacgctcctcctagagacttcgccgcctaccggtccagagtgaagttcagcagatccgccgatgctcccgcctatcagcagggacagaaccagctgtacaacgagctgaacctggggagaagagaagagtacgacgtgctggacaagcggagaggcagagatcctgagatgggcggcaagcccagacggaagaatcctcaagagggcctgtataatgagctgcagaaagacaagatggccgaggcctacagcgagatcggaatgaagggcgagcgcagaagaggcaagggacacgatggactgtaccagggcctgagcaccgccaccaaggatacctatgatgccctgcacatgcaggccctgcctccaaga

SEQ ID NO: 117 - DNA, 717 bp, synthetic construct
  source 1..717: mol_type = other DNA; note = nucleic acid encoding switchable chimeric antigen receptor
gagttcaagcctctgcctgaagtgaccgacgagtatggcggaagcggaggatctggcggatctaagccactgccagaagtcacagacgaatacgccgctgcaggcggttcaggcggatccgagtctaagtacggacctccttgtcctccatgtcctaccagaggcctggacttcgcctgcgacatctatatctgggcccctctggctggcacatgtggcgttttgctgctgagcctggtcatcaccctgtactgcaagcggggcagaaagaagctgctgtacatcttcaagcagcccttcatgcggcccgtgcagaccacacaagaggaagatggctgctcctgcagattccccgaggaagaagaaggcggctgcgagctgagagtgaagttcagcagatccgctgacgcccctgcctacaagcagggacagaaccagctgtacaacgagctgaacctggggagaagagaagagtacgacgtgctggacaagcggagaggcagagatcctgagatgggcggcaagcccagacggaagaatcctcaagagggcctgtataatgagctgcagaaagacaagatggccgaggcctacagcgagatcggaatgaagggcgagcgcagaagaggcaagggacacgatggactgtaccagggcctgagcaccgccaccaaggatacctatgatgccctgcacatgcaggccctgcctccaaga

SEQ ID NO: 118 - DNA, 774 bp, synthetic construct
  source 1..774: mol_type = other DNA; note = nucleic acid encoding switchable chimeric antigen receptor
gagttcaagcctctgcctgaagtgaccgacgagtatggcggaagcggaggatctggcggatctaagccactgccagaagtcacagacgaatacggcggttcaggtggcagcggaggctctaaacctcttccagaagttactgacgagtacgccgctgcaggcggttctggcggctctgagtctaagtacggacctccttgtcctccatgtcctaccagaggcctggacttcgcctgcgacatctatatctgggcccctctggctggcacatgtggcgttttgctgctgagcctggtcatcaccctgtactgcaagcggggcagaaagaagctgctgtacatcttcaagcagcccttcatgcggcccgtgcagaccacacaagaggaagatggctgctcctgcagattccccgaggaagaagaaggcggctgcgagctgagagtgaagttcagcagatccgctgacgcccctgcctacaagcagggacagaaccagctgtacaacgagctgaacctggggagaagagaagagtacgacgtgctggacaagcggagaggcagagatcctgagatgggcggcaagcccagacggaagaatcctcaagagggcctgtataatgagctgcagaaagacaagatggccgaggcctacagcgagatcggaatgaagggcgagcgcagaagaggcaagggacacgatggactgtaccagggcctgagcaccgccaccaaggatacctatgatgccctgcacatgcaggcccttccacctcgc

SEQ ID NO: 119 - DNA, 1041 bp, synthetic construct
  source 1..1041: mol_type = other DNA; note = nucleic acid encoding switchable chimeric antigen receptor
gagttcaagcctctgcctgaagtgaccgatgagtacgccgctgctggacctggtggcggaggatctaagattctggtcaagcagagccccatgctggtggcctacgacaacgccgtgaatctgagctgcaagtacagctacaacctgttcagcagagagttccgggccagcctgcacaaaggactggattctgctgtggaagtgtgcgtggtgtacggcaactacagccagcagctgcaggtctacagcaagaccggcttcaactgcgacggcaagctgggcaatgagagcgtgaccttctacctgcaaaacctgtacgtgaaccagaccgatatctacttctgcaagatcgaagtgatggcccctcctcctgctctggacaacgagaagtccaacggcaccatcatccacgtgaagggcaagcacctgtgtccttctccactgttccccggacctagcaagcctttctgggtgctcgttgttgttggcggcgtgctggcctgttatagcctgctggttaccgtggccttcatcatcttttgggtccgaagcaggcggagcagaggcggccacagcgactacatgaacatgacccctagacggcccggaccaaccagaaagcactaccagccttacgctcctcctagagacttcgccgcctacagatctggcggaggtggaagcggaggcggagcttcaggcggtggcggatcttttagcagatccgccgatgctcctgcctaccagcagggacagaaccagctgtacaacgagctgaacctggggagaagagaagagtacgatgtgctggacaggcggagaggcagagatcctgaaatgggcggcagacccagacggcggaatcctcaagagggcctgtataatgagctgcagcgcgacagaatggccgaggcctattctgagatcggcatgagaggcgagcggagaagaggtagaggacacgatggcctgtaccagggcctgagcacagccaccagagatacttatggcgccctgcacatgcaggccctgcctccaaga

SEQ ID NO: 120 - DNA, 1047 bp, synthetic construct
  source 1..1047: mol_type = other DNA; note = nucleic acid encoding switchable chimeric antigen receptor
gagttcagcaagcctctgcctgaagtgaccgacgagtacaagaatgccgccgctggtggatctggcggctctaagattctggtcaagcagagccctatgctggtggcctacgacaacgccgtgaacctgagctgcaagtacagctacaacctgttcagcagagagttccgggccagcctgcacaaaggactggattctgctgtggaagtgtgcgtggtgtacggcaactacagccagcagctgcaggtctacagcaagaccggcttcaactgcgacggcaagctgggcaatgagagcgtgaccttctacctgcaaaacctgtacgtgaaccagaccgatatctacttctgcaagatcgaagtgatggcccctcctcctgctctggacaacgagaagtccaacggcaccatcatccacgtgaagggcaagcacctgtgtccttctccactgttccccggacctagcaagcctttctgggtgctcgttgttgttggcggcgtgctggcctgttatagcctgctggttaccgtggccttcatcatcttttgggtccgaagcaagcggagcagaggcggccacagcgactacatgaacatgacccctagacggcccggaccaaccagaaagcactaccagccttacgctcctcctagagacttcgccgcctatagaagcggaggcggaggttctggtggcggtgcttctggcggcggaggaagcttttccagatctgccgatgctcccgcctatcagcagggccagaaccagctgtacaacgagctgaacctggggagaagagaagagtacgacgtgctggacaagcggagaggcagagatcctgagatgggcggcaagcccagacggaagaatcctcaagagggcctgtacaatgaactgcagaaagacaagatggccgaggcctacagcgagatcggaatgaagggcgagcgcagaagaggcaagggacacgatggactgtaccagggcctgagcacagccaccaaggatacttatggcgccctgcacatgcaggccctgcctccaaga

SEQ ID NO: 121 - DNA, 609 bp, synthetic construct
  source 1..609: mol_type = other DNA; note = nucleic acid encoding switchable chimeric antigen receptor
gagttcaagcctctgcctgaagtgaccgacgagtacgagtctaagtacggccctccttgtcctccatgtcctgacatctacatctgggcccctctggccggaacatgtggtgttctgctgctgagcctggtcatcaccctgtactgcaagcggggcagaaagaagctgctgtacatcttcaagcagcccttcatgcggcccgtgcagaccacacaagaggaagatggctgctcctgcagattccccgaggaagaagaaggcggctgcgagctgagagtgaagttcagcagatccgccgacgctcctgcctatcagcagggacagaaccagctgtacaacgagctgaacctggggagaagagaagagtacgacgtgctggacaagcggagaggcagagatcctgagatgggcggcaagcccagacggaagaatcctcaagagggcctgtataatgagctgcagaaagacaagatggccgaggcctacagcgagatcggaatgaagggcgagcgcagaagaggcaagggacacgatggactgtaccagggcctgagcaccgccaccaaggatacctatgatgccctgcacatgcaggccctgcctccaaga

SEQ ID NO: 122 - DNA, 618 bp, synthetic construct
  source 1..618: mol_type = other DNA; note = nucleic acid encoding switchable chimeric antigen receptor
gagttcaagcctctgcctgaagtgaccgacgagtatgccgccgctgagtctaagtacggccctccttgtcctccatgtcctgacatctacatctgggcccctctggccggaacatgtggtgttctgctgctgagcctggtcatcaccctgtactgcaagcggggcagaaagaagctgctgtacatcttcaagcagcccttcatgcggcccgtgcagaccacacaagaggaagatggctgctcctgcagattccccgaggaagaagaaggcggctgcgagctgagagtgaagttcagcagatccgccgacgctcctgcctatcagcagggacagaaccagctgtacaacgagctgaacctggggagaagagaagagtacgacgtgctggacaagcggagaggcagagatcctgagatgggcggcaagcccagacggaagaatcctcaagagggcctgtataatgagctgcagaaagacaagatggccgaggcctacagcgagatcggaatgaagggcgagcgcagaagaggcaagggacacgatggactgtaccagggcctgagcaccgccaccaaggatacctatgatgccctgcacatgcaggccctgcctccaaga

SEQ ID NO: 123 - DNA, 636 bp, synthetic construct
  source 1..636: mol_type = other DNA; note = nucleic acid encoding switchable chimeric antigen receptor
gagttcaagcctctgcctgaagtgaccgatgagtatgccgctgctggtggatctggcggcagcgagtctaagtacggacctccttgtcctccatgtcctgacatctacatctgggcccctctggccggaacatgtggtgttctgctgctgagcctggtcatcaccctgtactgcaagcggggcagaaagaagctgctgtacatcttcaagcagcccttcatgcggcccgtgcagaccacacaagaggaagatggctgctcctgcagattccccgaggaagaagaaggcggctgcgagctgagagtgaagttcagcagatccgccgacgctcctgcctatcagcagggacagaaccagctgtacaacgagctgaacctggggagaagagaagagtacgacgtgctggacaagcggagaggcagagatcctgagatgggcggcaagcccagacggaagaatcctcaagagggcctgtataatgagctgcagaaagacaagatggccgaggcctacagcgagatcggaatgaagggcgagcgcagaagaggcaagggacacgatggactgtaccagggcctgagcaccgccaccaaggatacctatgatgccctgcacatgcaggccctgcctccaaga

SEQ ID NO: 124 - DNA, 621 bp, synthetic construct
  source 1..621: mol_type = other DNA; note = nucleic acid encoding switchable chimeric antigen receptor
agcaagcccctgcctgaagtgaccgacgagtacaagaatgccgccgctgagtctaagtacggccctccttgtcctccatgtcctgacatctatatctgggcccctctggccggaacatgtggcgttttgctgctgagcctggtcatcaccctgtactgcaagcggggcagaaagaagctgctgtacatcttcaagcagcccttcatgcggcccgtgcagaccacacaagaggaagatggctgctcctgcagattccccgaggaagaagaaggcggctgcgagctgagagtgaagttcagcagatccgccgacgctcctgcctatcagcagggacagaaccagctgtacaacgagctgaacctggggagaagagaagagtacgacgtgctggacaagcggagaggcagagatcctgagatgggcggcaagcccagacggaagaatcctcaagagggcctgtataatgagctgcagaaagacaagatggccgaggcctacagcgagatcggaatgaagggcgagcgcagaagaggcaagggacacgatggactgtaccagggcctgagcaccgccaccaaggatacctatgatgccctgcacatgcaggccctgcctccaaga

SEQ ID NO: 125 - DNA, 1119 bp, synthetic construct
  source 1..1119: mol_type = other DNA; note = nucleic acid encoding switchable chimeric antigen receptor
gagaacggcgacaacgagaaaatggccgctctggaagccaagatctgccaccagatcgagtactacttcggcgacttcaacctgcctcgggacaagttcctgaaagagcagatcaagctggacgaaggctgggtgcccctggaaatcatgatcaagttcaaccggctgaacaggctgaccaccgacttcaatgtgatcgtggaagccctgagcaagagcaaggccgagctgatggaaatcagcgaggacaagaccaagatccggcggagcccttctaagcccctgcctgaagtgaccgacgagtacaagaacgacgtgaagaaccgcagcgtgtacatcaagggcttccccaccgatgccacactggacgacatcaaagagtggcttgaggacaaaggccaggtgctgaacatccagatgcggcggacactgcacaaggccttcaagggcagcatcttcgtggtgttcgacagcatcgagagcgccaagaaattcgtggaaacccctggccagaagtacaaagagacagacctgctgatcctgttcgagtctaagtacggccctccttgtcctccatgtcctgacatctacatctgggcccctctggccggaacatgtggtgttctgctgctgagcctggtcatcaccctgtactgcaagcggggcagaaagaagctgctgtacatcttcaagcagcccttcatgcggcccgtgcagaccacacaagaggaagatggctgctcctgcagattccccgaggaagaagaaggcggctgcgagctgagagtgaagttcagcagatccgccgacgctcctgcctatcagcagggacagaaccagctgtacaacgagctgaacctggggagaagagaagagtacgacgtgctggacaagcggagaggcagagatcctgagatgggcggcaagcccagacggaagaatcctcaagagggcctgtataatgagctgcagaaagacaagatggccgaggcctacagcgagatcggaatgaagggcgagcgcagaagaggcaagggacacgatggactgtaccagggcctgagcaccgccaccaaggatacctatgatgccctgcacatgcaggccctgcctccaaga

SEQ ID NO: 126 - DNA, 661 bp, synthetic construct
  source 1..661: mol_type = other DNA; note = nucleic acid encoding switchable chimeric antigen receptor
gagttcaagcctctgcctgaagtgaccgacgagtatggcggcggaggcagcgagtttaaacccctgccagaagtcacagacgaatacgagtctaagtacggccctccttgtcctccatgtcctgacatctacatctgggcccctctggccggaacatgtggtgttctgctgctgagcctggtcatcaccctgtactgcaagcggggcagaaagaagctgctgtacatcttcaagcagcccttcatgcggcccgtgcagaccacacaagaggaagatggctgctcctgcagattccccgaggaagaagaaggcggctgcgagctgagagtgaagttcagcagatccgccgacgctcctgcctatcagcagggacagaaccagctgtacaacgagctgaacctggggagaagagaagagtacgacgtgctggacaagcggagaggcagagatcctgagatgggcggcaagcccagacggaagaatcctcaagagggcctgtataatgagctgcagaaagacaagatggccgaggcctacagcgagatcggaatgaagggcgagcgcagaagaggcaagggacacgatggactgtaccagggcctgagcaccgccaccaaggatacctatgatgccctgcacatgcaggccctgcctccaagag

SEQ ID NO: 127 - DNA, 624 bp, synthetic construct
  source 1..624: mol_type = other DNA; note = nucleic acid encoding switchable chimeric antigen receptor
gagttcaagcctctgcctgaagtgaccgacgagtatgccgccgctgagtctaagtacggccctccttgtcctccatgtcctatgttctgggtgctcgtggttgttggcggagtgctggcctgttacagcctgctggttaccgtggccttcatcatcttttgggtccgaagcaagcggagccggctgctgcacagcgactacatgaacatgacccctagacggcccggacctaccagaaagcactaccagccttacgctcctcctagagacttcgccgcctaccggtccagagtgaagttcagcagatccgccgatgctcccgcctatcagcagggacagaaccagctgtacaacgagctgaacctggggagaagagaagagtacgacgtgctggacaagcggagaggcagagatcctgagatgggcggcaagcccagacggaagaatcctcaagagggcctgtataatgagctgcagaaagacaagatggccgaggcctacagcgagatcggaatgaagggcgagcgcagaagaggcaagggacacgatggactgtaccagggactgagcaccgccaccaaggatacctatgacgccctgcacatgcaggccctgcctccaaga

SEQ ID NO: 128 - DNA, 627 bp, synthetic construct
  source 1..627: mol_type = other DNA; note = nucleic acid encoding switchable chimeric antigen receptor
gagttcaagcctctgcctgaagtgaccgacgagtatgccgccgctgagtctaagtacggccctccttgtcctccatgtcctatgttctgggtgctcgtggttgttggcggagtgctggcctgttacagcctgctggttaccgtggccttcatcatcttttgggtcaagcggggcagaaagaagctgctgtacatcttcaagcagcccttcatgcggcccgtgcagaccacacaagaggaagatggctgctcctgcagattccccgaggaagaagaaggcggctgcgagctgagagtgaagttcagcagatccgccgacgctcctgcctatcagcagggacagaaccagctgtacaacgagctgaacctggggagaagagaagagtacgacgtgctggacaagcggagaggcagagatcctgagatgggcggcaagcccagacggaagaatcctcaagagggcctgtataatgagctgcagaaagacaagatggccgaggcctacagcgagatcggaatgaagggcgagcgcagaagaggcaagggacacgatggactgtaccagggactgagcaccgccaccaaggatacctatgacgccctgcacatgcaggccctgcctccaaga

SEQ ID NO: 129 - DNA, 666 bp, synthetic construct
  source 1..666: mol_type = other DNA; note = nucleic acid encoding switchable chimeric antigen receptor
gagttcaagcctctgcctgaagtgaccgacgagtatggcggcggaggcagcgagtttaaacccctgccagaagtcacagacgaatacgagtctaagtacggccctccttgtcctccatgtcctatgttctgggtgctcgtggttgttggcggagtgctggcctgttacagcctgctggttaccgtggccttcatcatcttttgggtccgaagcaagcggagccggctgctgcacagcgactacatgaacatgacccctagacggcccggacctaccagaaagcactaccagccttacgctcctcctagagacttcgccgcctaccggtccagagtgaagttcagcagatccgccgatgctcccgcctatcagcagggacagaaccagctgtacaacgagctgaacctggggagaagagaagagtacgacgtgctggacaagcggagaggcagagatcctgagatgggcggcaagcccagacggaagaatcctcaagagggcctgtataatgagctgcagaaagacaagatggccgaggcctacagcgagatcggaatgaagggcgagcgcagaagaggcaagggacacgatggactgtaccagggactgagcaccgccaccaaggatacctatgacgccctgcacatgcaggccctgcctccaaga

SEQ ID NO: 130 - DNA, 666 bp, synthetic construct
  source 1..666: mol_type = other DNA; note = nucleic acid encoding switchable chimeric antigen receptor
gagttcaagcctctgcctgaagtgaccgacgagtatggcggcggaggcagcgagtttaaacccctgccagaagtcacagacgaatacgagtctaagtacggccctccttgtcctccatgtcctatgttctgggtgctcgtggttgttggcggagtgctggcctgttacagcctgctggttaccgtggccttcatcatcttttgggtccgaagcaagcggagcagaggcggccacagcgactacatgaacatgacccctagacggcccggacctaccagaaagcactaccagccttacgctcctcctagagacttcgccgcctaccggtccagagtgaagttcagcagatccgccgatgctcccgcctatcagcagggacagaaccagctgtacaacgagctgaacctggggagaagagaagagtacgacgtgctggacaagcggagaggcagagatcctgagatgggcggcaagcccagacggaagaatcctcaagagggcctgtataatgagctgcagaaagacaagatggccgaggcctacagcgagatcggaatgaagggcgagcgcagaagaggcaagggacacgatggactgtaccagggactgagcaccgccaccaaggatacctatgacgccctgcacatgcaggccctgcctccaaga

SEQ ID NO: 131 - DNA, 657 bp, synthetic construct
  source 1..657: mol_type = other DNA; note = nucleic acid encoding switchable chimeric antigen receptor
gagttcaagcctctgcctgaagtgaccgacgagtatggcggcggaggcagcgagtttaaacccctgccagaagtcacagacgaatacgagtctaagtacggccctccttgtcctccatgtcctgacatctacatctgggcccctctggccggaacatgtggtgttctgctgctgagcctggtcatcaccctgtactgcagaagcaagagaagcagaggcggccacagcgactacatgaacatgacccctagacggcccggacctaccagaaagcactaccagccttacgctcctcctagagacttcgccgcctaccggtccagagtgaagttcagcagatccgccgatgctcccgcctatcagcagggacagaaccagctgtacaacgagctgaacctggggagaagagaagagtacgacgtgctggacaagcggagaggcagagatcctgagatgggcggcaagcccagacggaagaatcctcaagagggcctgtataatgagctgcagaaagacaagatggccgaggcctacagcgagatcggaatgaagggcgaacgcagaagaggcaagggccacgatggactgtatcagggcctgagcaccgccaccaaggatacctatgatgccctgcacatgcaggccctgcctccaaga

SEQ ID NO: 132 - DNA, 669 bp, synthetic construct
  source 1..669: mol_type = other DNA; note = nucleic acid encoding switchable chimeric antigen receptor
gagttcaagcctctgcctgaagtgaccgacgagtatggcggcggaggcagcgagtttaaacccctgccagaagtcacagacgaatacgagtctaagtacggccctccttgtcctccatgtcctatgttctgggtgctcgtggttgttggcggagtgctggcctgttacagcctgctggttaccgtggccttcatcatcttttgggtcaagcggggcagaaagaagctgctgtacatcttcaagcagcccttcatgcggcccgtgcagaccacacaagaggaagatggctgctcctgcagattccccgaggaagaagaaggcggctgcgagctgagagtgaagttcagcagatccgccgacgctcctgcctatcagcagggacagaaccagctgtacaacgagctgaacctggggagaagagaagagtacgacgtgctggacaagcggagaggcagagatcctgagatgggcggcaagcccagacggaagaatcctcaagagggcctgtataatgagctgcagaaagacaagatggccgaggcctacagcgagatcggaatgaagggcgagcgcagaagaggcaagggacacgatggactgtaccagggactgagcaccgccaccaaggatacctatgacgccctgcacatgcaggccctgcctccaaga

SEQ ID NO: 133 - DNA, 669 bp, synthetic construct
  source 1..669: mol_type = other DNA; note = nucleic acid encoding switchable chimeric antigen receptor
gagttcaagcctctgcctgaagtgaccgacgagtatggcggcggaggcagcgagtttaaacccctgccagaagtcacagacgaatacgagtctaagtacggccctccttgtcctccatgtcctatgttctgggtgctcgtggttgttggcggagtgctggcctgttacagcctgctggttaccgtggccttcatcatcttttgggtcaagcggggcagaaagaaaggcggctacatcttcaagcagcccttcatgaggcccgtgcagaccacacaagaggaagatggctgctcctgcagattccccgaggaagaagaaggcggctgcgagctgagagtgaagttcagcagatccgccgacgctcctgcctatcagcagggacagaaccagctgtacaacgagctgaacctggggagaagagaagagtacgacgtgctggacaagcggagaggcagagatcctgagatgggcggcaagcccagacggaagaatcctcaagagggcctgtataatgagctgcagaaagacaagatggccgaggcctacagcgagatcggaatgaagggcgagcgcagaagaggcaagggacacgatggactgtaccagggactgagcaccgccaccaaggatacctatgacgccctgcacatgcaggccctgcctccaaga

SEQ ID NO: 134 - DNA, 642 bp, synthetic construct
  source 1..642: mol_type = other DNA; note = nucleic acid encoding switchable chimeric antigen receptor
gagttcaagcctctgcctgaagtgaccgatgagtatgccgctgctggtggatctggcggcagcgagtctaagtacggacctccttgtcctccatgtcctatgttctgggtgctcgtggttgttggcggagtgctggcctgttacagcctgctggttaccgtggccttcatcatcttttgggtccgaagcaagcggagccggctgctgcacagcgactacatgaacatgacccctagacggcccggacctaccagaaagcactaccagccttacgctcctcctagagacttcgccgcctaccggtccagagtgaagttcagcagatccgccgatgctcccgcctatcagcagggacagaaccagctgtacaacgagctgaacctggggagaagagaagagtacgacgtgctggacaagcggagaggcagagatcctgagatgggcggcaagcccagacggaagaatcctcaagagggcctgtataatgagctgcagaaagacaagatggccgaggcctacagcgagatcggaatgaagggcgagcgcagaagaggcaagggacacgatggactgtaccagggactgagcaccgccaccaaggatacctatgacgccctgcacatgcaggccctgcctccaaga

SEQ ID NO: 135 - DNA, 642 bp, synthetic construct
  source 1..642: mol_type = other DNA; note = nucleic acid encoding switchable chimeric antigen receptor
gagttcaagcctctgcctgaagtgaccgatgagtatgccgctgctggtggatctggcggcagcgagtctaagtacggacctccttgtcctccatgtcctatgttctgggtgctcgtggttgttggcggagtgctggcctgttacagcctgctggttaccgtggccttcatcatcttttgggtccgaagcaagcggagcagaggcggccacagcgactacatgaacatgacccctagacggcccggacctaccagaaagcactaccagccttacgctcctcctagagacttcgccgcctaccggtccagagtgaagttcagcagatccgccgatgctcccgcctatcagcagggacagaaccagctgtacaacgagctgaacctggggagaagagaagagtacgacgtgctggacaagcggagaggcagagatcctgagatgggcggcaagcccagacggaagaatcctcaagagggcctgtataatgagctgcagaaagacaagatggccgaggcctacagcgagatcggaatgaagggcgagcgcagaagaggcaagggacacgatggactgtaccagggactgagcaccgccaccaaggatacctatgacgccctgcacatgcaggccctgcctccaaga

SEQ ID NO: 136 - DNA, 633 bp, synthetic construct
  source 1..633: mol_type = other DNA; note = nucleic acid encoding switchable chimeric antigen receptor
gagttcaagcctctgcctgaagtgaccgatgagtatgccgctgctggtggatctggcggcagcgagtctaagtacggacctccttgtcctccatgtcctgacatctacatctgggcccctctggccggaacatgtggtgttctgctgctgagcctggtcatcaccctgtactgcagaagcaagagaagcagaggcggccacagcgactacatgaacatgacccctagacggcccggacctaccagaaagcactaccagccttacgctcctcctagagacttcgccgcctaccggtccagagtgaagttcagcagatccgccgatgctcccgcctatcagcagggacagaaccagctgtacaacgagctgaacctggggagaagagaagagtacgacgtgctggacaagcggagaggcagagatcctgagatgggcggcaagcccagacggaagaatcctcaagagggcctgtataatgagctgcagaaagacaagatggccgaggcctacagcgagatcggaatgaagggcgaacgcagaagaggcaagggccacgatggactgtatcagggcctgagcaccgccaccaaggatacctatgatgccctgcacatgcaggccctgcctccaaga

SEQ ID NO: 137 - DNA, 645 bp, synthetic construct
  source 1..645: mol_type = other DNA; note = nucleic acid encoding switchable chimeric antigen receptor
gagttcaagcctctgcctgaagtgaccgatgagtatgccgctgctggtggatctggcggcagcgagtctaagtacggacctccttgtcctccatgtcctatgttctgggtgctcgtggttgttggcggagtgctggcctgttacagcctgctggttaccgtggccttcatcatcttttgggtcaagcggggcagaaagaagctgctgtacatcttcaagcagcccttcatgcggcccgtgcagaccacacaagaggaagatggctgctcctgcagattccccgaggaagaagaaggcggctgcgagctgagagtgaagttcagcagatccgccgacgctcctgcctatcagcagggacagaaccagctgtacaacgagctgaacctggggagaagagaagagtacgacgtgctggacaagcggagaggcagagatcctgagatgggcggcaagcccagacggaagaatcctcaagagggcctgtataatgagctgcagaaagacaagatggccgaggcctacagcgagatcggaatgaagggcgagcgcagaagaggcaagggacacgatggactgtaccagggactgagcaccgccaccaaggatacctatgacgccctgcacatgcaggccctgcctccaaga

SEQ ID NO: 138 - DNA, 645 bp, synthetic construct
  source 1..645: mol_type = other DNA; note = nucleic acid encoding switchable chimeric antigen receptor
gagttcaagcctctgcctgaagtgaccgatgagtatgccgctgctggtggctctggcggcagcgagtctaaatacggacctccttgtcctccatgtcctatgttctgggtgctcgtggttgttggcggagtgctggcctgttacagcctgctggttaccgtggccttcatcatcttttgggtcaagcggggcagaaagaaaggcggctacatcttcaagcagcccttcatgaggcccgtgcagaccacacaagaggaagatggctgctcctgcagattccccgaggaagaagaaggcggctgcgagctgagagtgaagttcagcagatccgccgacgctcctgcctatcagcagggacagaaccagctgtacaacgagctgaacctggggagaagagaagagtacgacgtgctggacaagcggagaggcagagatcctgagatgggcggcaagcccagacggaagaatcctcaagagggcctgtataatgagctgcagaaagacaagatggccgaggcctacagcgagatcggaatgaagggcgagcgcagaagaggcaagggacacgatggactgtaccagggactgagcaccgccaccaaggatacctatgacgccctgcacatgcaggccctgcctccaaga

SEQ ID NO: 139 - DNA, 738 bp, synthetic construct
  source 1..738: mol_type = other DNA; note = nucleic acid encoding switchable chimeric antigen receptor
gagtttaaaccactgcctgaggtgaccgatgagtacggcggcggcggcagcgagttcaagcccctgcctgaggtgactgatgagtatatcgaagtgatgtaccctcccccctatctggacaacgaaaaatctaacggcaccatcatccacgtcaaaggcaaacacctgtgcccatccccactgttccctggcccatctaagcccgacatctacatctgggcccctctggccggcacatgcggcgtgctgctgctcagcctggtgattacactgtactgccggtccaagagatccaggggcggccactctgactacatgaacatgacccccaggagacccggccccaccaggaaacactaccagccctacgcccccccccgggattttgccgcttaccgctccagggtgaagtttagcagatccgctgatgcccctgcctatcagcagggacagaaccagctgtacaacgagctgaacctggggagaagagaagagtacgatgtgctggacaagcggagaggcagagatcctgagatgggcggcaagcccagacggaagaatcctcaagagggcctgtacaatgaactgcagaaagacaagatggccgaggcctacagcgagatcggaatgaagggcgagcgcagaagaggcaagggacacgatggactgtaccagggcctgagcaccgccaccaaggatacctatgatgccctgcacatgcaggccctgcctccaaga

SEQ ID NO: 140 - DNA, 615 bp, synthetic construct
  source 1..615: mol_type = other DNA; note = nucleic acid encoding switchable chimeric antigen receptor
gagttcaagcctctgcctgaagtgaccgacgagtacgagtctaagtacggccctccttgtcctccatgtcctatgttctgggtgctcgtggttgttggcggagtgctggcctgttacagcctgctggttaccgtggccttcatcatcttttgggtccgaagcaagcggagcagaggcggccacagcgactacatgaacatgacccctagacggcccggacctaccagaaagcactaccagccttacgctcctcctagagacttcgccgcctaccggtccagagtgaagttcagcagatccgccgatgctcccgcctatcagcagggacagaaccagctgtacaacgagctgaacctggggagaagagaagagtacgacgtgctggacaagcggagaggcagagatcctgagatgggcggcaagcccagacggaagaatcctcaagagggcctgtataatgagctgcagaaagacaagatggccgaggcctacagcgagatcggaatgaagggcgagcgcagaagaggcaagggacacgatggactgtaccagggactgagcaccgccaccaaggatacctatgacgccctgcacatgcaggccctgcctccaaga

SEQ ID NO: 141 - DNA, 618 bp, synthetic construct
  source 1..618: mol_type = other DNA; note = nucleic acid encoding switchable chimeric antigen receptor
gagttcaagcctctgcctgaagtgaccgacgagtacgagtctaagtacggccctccttgtcctccatgtcctatgttctgggtgctcgtggttgttggcggagtgctggcctgttacagcctgctggttaccgtggccttcatcatcttttgggtcaagcggggcagaaagaaaggcggctacatcttcaagcagcccttcatgaggcccgtgcagaccacacaagaggaagatggctgctcctgcagattccccgaggaagaagaaggcggctgcgagctgagagtgaagttcagcagatccgccgacgctcctgcctatcagcagggacagaaccagctgtacaacgagctgaacctggggagaagagaagagtacgacgtgctggacaagcggagaggcagagatcctgagatgggcggcaagcccagacggaagaatcctcaagagggcctgtataatgagctgcagaaagacaagatggccgaggcctacagcgagatcggaatgaagggcgagcgcagaagaggcaagggacacgatggactgtaccagggactgagcaccgccaccaaggatacctatgacgccctgcacatgcaggccctgcctccaaga

SEQ ID NO: 142 - DNA, 636 bp, synthetic construct; identical to SEQ ID NO: 123
  source 1..636: mol_type = other DNA; note = nucleic acid encoding switchable chimeric antigen receptor

SEQ ID NO: 143 - protein, 231 aa, synthetic construct
  source 1..231: note = silenced IgG1 Fc-knob
EPKSCDKTHTCPPCPAPPVAGPSVFLFPPKPKDTLMISRTPEVTCVVVDVSHEDPEVKFNWYVDGVEVHNAKTKPREEQYNSTYRVVSVLTVLHQDWLNGKEYKCKVSNKGLPSSIEKTISKAKGQPREPQVYTLPPSRDELTKNQVSLWCLVKGFYPSDIAVEWESNGQPENNYKTTPPVLDSDGSFFLYSKLTVDKSRWQQGNVFSCSVMHEALHNHYTQKSLSLSPGK

SEQ ID NO: 144 - protein, 231 aa, synthetic construct
  source 1..231: note = silenced IgG1 Fc-hole
EPKSCDKTHTCPPCPAPPVAGPSVFLFPPKPKDTLMISRTPEVTCVVVDVSHEDPEVKFNWYVDGVEVHNAKTKPREEQYNSTYRVVSVLTVLHQDWLNGKEYKCKVSNKGLPSSIEKTISKAKGQPREPQVYTLPPSRDELTKNQVSLSCAVKGFYPSDIAVEWESNGQPENNYKTTPPVLDSDGSFFLVSKLTVDKSRWQQGNVFSCSVMHEALHNHYTQKSLSLSPGK

SEQ ID NO: 145 - protein, 22 aa, Homo sapiens
MDMRAPAQVFGFLLLWFPGARC

SEQ ID NO: 146 - protein, 19 aa, Mus musculus
MGWSCIILFLVATATGVHS

SEQ ID NO: 147 - protein, 450 aa, synthetic construct
  source 1..450: note = targeting module chain
GQVQLVQSGAEVKKPGASVKVSCKASGYTFTHYYIYWVRQAPGQGLEWMGGVNPSNGGTHFNEKFKSRVTMTRDTSISTAYMELSRLRSDDTAVYYCARSEYDYGLGFAYWGQGTLVTVSSASTKGPSVFPLAPSSKSTSGGTAALGCLVKDYFPEPVTVSWNSGALTSGVHTFPAVLQSSGLYSLSSVVTVPSSSLGTQTYICNVNHKPSNTKVDKKVEPKSCDKTHTCPPCPAPPVAGPSVFLFPPKPKDTLMISRTPEVTCVVVDVSHEDPEVKFNWYVDGVEVHNAKTKPREEQYNSTYRVVSVLTVLHQDWLNGKEYKCKVSNKGLPSSIEKTISKAKGQPREPQVYTLPPSRDELTKNQVSLWCLVKGFYPSDIAVEWESNGQPENNYKTTPPVLDSDGSFFLYSKLTVDKSRWQQGNVFSCSVMHEALHNHYTQKSLSLSPGK

SEQ ID NO: 148 - protein, 469 aa, synthetic construct
  source 1..469: note = targeting module chain
MGWSCIILFLVATATGVHSGQVQLVQSGAEVKKPGASVKVSCKASGYTFTHYYIYWVRQAPGQGLEWMGGVNPSNGGTHFNEKFKSRVTMTRDTSISTAYMELSRLRSDDTAVYYCARSEYDYGLGFAYWGQGTLVTVSSASTKGPSVFPLAPSSKSTSGGTAALGCLVKDYFPEPVTVSWNSGALTSGVHTFPAVLQSSGLYSLSSVVTVPSSSLGTQTYICNVNHKPSNTKVDKKVEPKSCDKTHTCPPCPAPPVAGPSVFLFPPKPKDTLMISRTPEVTCVVVDVSHEDPEVKFNWYVDGVEVHNAKTKPREEQYNSTYRVVSVLTVLHQDWLNGKEYKCKVSNKGLPSSIEKTISKAKGQPREPQVYTLPPSRDELTKNQVSLWCLVKGFYPSDIAVEWESNGQPENNYKTTPPVLDSDGSFFLYSKLTVDKSRWQQGNVFSCSVMHEALHNHYTQKSLSLSPGK

SEQ ID NO: 149 - protein, 350 aa, synthetic construct
  source 1..350: note = targeting module chain
DIVMTQSPDSLAVSLGERATINCKSSQSLLNSRTPKNYLAWYQQKPGQPPKLLIYWASTRKSGVPDRFSGSGSGTDFTLTISSLQAEDVAVYYCKQSYNLLTFGGGTKVEIKRTVAAPSVFIFPPSDEQLKSGTASVVCLLNNFYPREAKVQWKVDNALQSGNSQESVTEQDSKDSTYSLSSTLTLSKADYEKHKVYACEVTHQGLSSPVTKSFNRGECGGGGSGGGGSGGGGSEVQLVESGGGLVQPGGSLRLSCAASGFSFSDFWMSWVRQAPGKGLEWVATISQAGSEKDYVDSVKGRFTISRDNAKKSLYLQMNSLRAEDTAVYYCASGVYSFDYRGQGTLVTVSS

SEQ ID NO: 150 - protein, 372 aa, synthetic construct
  source 1..372: note = targeting module chain
MDMRAPAQVFGFLLLWFPGARCDIVMTQSPDSLAVSLGERATINCKSSQSLLNSRTPKNYLAWYQQKPGQPPKLLIYWASTRKSGVPDRFSGSGSGTDFTLTISSLQAEDVAVYYCKQSYNLLTFGGGTKVEIKRTVAAPSVFIFPPSDEQLKSGTASVVCLLNNFYPREAKVQWKVDNALQSGNSQESVTEQDSKDSTYSLSSTLTLSKADYEKHKVYACEVTHQGLSSPVTKSFNRGECGGGGSGGGGSGGGGSEVQLVESGGGLVQPGGSLRLSCAASGFSFSDFWMSWVRQAPGKGLEWVATISQAGSEKDYVDSVKGRFTISRDNAKKSLYLQMNSLRAEDTAVYYCASGVYSFDYRGQGTLVTVSS

SEQ ID NO: 151 - protein, 353 aa, synthetic construct
  source 1..353: note = targeting module chain
GQVQLQESGGGLVQAGGSLRLSCAASGRTFSNYNMGWFRQAPGKEREFVAAIDWSGGSPYYAASVRGRFTISRDNAENTVYLQMNSLKPEDTAVYYCAAPLSYGSTWLADYWGQGTQVTVSSEPKSCDKTHTCPPCPAPPVAGPSVFLFPPKPKDTLMISRTPEVTCVVVDVSHEDPEVKFNWYVDGVEVHNAKTKPREEQYNSTYRVVSVLTVLHQDWLNGKEYKCKVSNKGLPSSIEKTISKAKGQPREPQVYTLPPSRDELTKNQVSLSCAVKGFYPSDIAVEWESNGQPENNYKTTPPVLDSDGSFFLVSKLTVDKSRWQQGNVFSCSVMHEALHNHYTQKSLSLSPGK

SEQ ID NO: 152 - protein, 372 aa, synthetic construct
  source 1..372: note = targeting module chain
MGWSCIILFLVATATGVHSGQVQLQESGGGLVQAGGSLRLSCAASGRTFSNYNMGWFRQAPGKEREFVAAIDWSGGSPYYAASVRGRFTISRDNAENTVYLQMNSLKPEDTAVYYCAAPLSYGSTWLADYWGQGTQVTVSSEPKSCDKTHTCPPCPAPPVAGPSVFLFPPKPKDTLMISRTPEVTCVVVDVSHEDPEVKFNWYVDGVEVHNAKTKPREEQYNSTYRVVSVLTVLHQDWLNGKEYKCKVSNKGLPSSIEKTISKAKGQPREPQVYTLPPSRDELTKNQVSLSCAVKGFYPSDIAVEWESNGQPENNYKTTPPVLDSDGSFFLVSKLTVDKSRWQQGNVFSCSVMHEALHNHYTQKSLSLSPGK

SEQ ID NO: 153 - protein, 353 aa, synthetic construct
  source 1..353: note = targeting module chain
GQVQLVESGGGLVQPGGSLRLSCAASGRTFSNYNMGWFRQAPGQGLEFVAAIDWSGGSPYYADSVKGRFTISRDNSKNTLYLQMNSLRAEDTAVYYCAAPLSYGSTWLADYWGQGTLVTVSSEPKSCDKTHTCPPCPAPPVAGPSVFLFPPKPKDTLMISRTPEVTCVVVDVSHEDPEVKFNWYVDGVEVHNAKTKPREEQYNSTYRVVSVLTVLHQDWLNGKEYKCKVSNKGLPSSIEKTISKAKGQPREPQVYTLPPSRDELTKNQVSLSCAVKGFYPSDIAVEWESNGQPENNYKTTPPVLDSDGSFFLVSKLTVDKSRWQQGNVFSCSVMHEALHNHYTQKSLSLSPGK

SEQ ID NO: 154 - protein, 372 aa, synthetic construct
  source 1..372: note = targeting module chain
MGWSCIILFLVATATGVHSGQVQLVESGGGLVQPGGSLRLSCAASGRTFSNYNMGWFRQAPGQGLEFVAAIDWSGGSPYYADSVKGRFTISRDNSKNTLYLQMNSLRAEDTAVYYCAAPLSYGSTWLADYWGQGTLVTVSSEPKSCDKTHTCPPCPAPPVAGPSVFLFPPKPKDTLMISRTPEVTCVVVDVSHEDPEVKFNWYVDGVEVHNAKTKPREEQYNSTYRVVSVLTVLHQDWLNGKEYKCKVSNKGLPSSIEKTISKAKGQPREPQVYTLPPSRDELTKNQVSLSCAVKGFYPSDIAVEWESNGQPENNYKTTPPVLDSDGSFFLVSKLTVDKSRWQQGNVFSCSVMHEALHNHYTQKSLSLSPGK

SEQ ID NO: 155 - protein, 353 aa, synthetic construct
  source 1..353: note = targeting module chain
GQVQLVESGGGLVQPGGSLRLSCAASGRTFSNYNMGWFRQAPGQGLEFVAAIDWSGGSPYYAASVRGRFTISRDNSKNTLYLQMNSLRAEDTAVYYCAAPLSYGSTWLADYWGQGTLVTVSSEPKSCDKTHTCPPCPAPPVAGPSVFLFPPKPKDTLMISRTPEVTCVVVDVSHEDPEVKFNWYVDGVEVHNAKTKPREEQYNSTYRVVSVLTVLHQDWLNGKEYKCKVSNKGLPSSIEKTISKAKGQPREPQVYTLPPSRDELTKNQVSLSCAVKGFYPSDIAVEWESNGQPENNYKTTPPVLDSDGSFFLVSKLTVDKSRWQQGNVFSCSVMHEALHNHYTQKSLSLSPGK

SEQ ID NO: 156 - protein, 372 aa, synthetic construct
  source 1..372: note = targeting module chain
MGWSCIILFLVATATGVHSGQVQLVESGGGLVQPGGSLRLSCAASGRTFSNYNMGWFRQAPGQGLEFVAAIDWSGGSPYYAASVRGRFTISRDNSKNTLYLQMNSLRAEDTAVYYCAAPLSYGSTWLADYWGQGTLVTVSSEPKSCDKTHTCPPCPAPPVAGPSVFLFPPKPKDTLMISRTPEVTCVVVDVSHEDPEVKFNWYVDGVEVHNAKTKPREEQYNSTYRVVSVLTVLHQDWLNGKEYKCKVSNKGLPSSIEKTISKAKGQPREPQVYTLPPSRDELTKNQVSLSCAVKGFYPSDIAVEWESNGQPENNYKTTPPVLDSDGSFFLVSKLTVDKSRWQQGNVFSCSVMHEALHNHYTQKSLSLSPGK

SEQ ID NO: 157 - protein, 484 aa, synthetic construct
  source 1..484: note = targeting module chain
GQVQLQESGGGLVQAGGSLRLSCAASGRTFSNYNMGWFRQAPGKEREFVAAIDWSGGSPYYAASVRGRFTISRDNAENTVYLQMNSLKPEDTAVYYCAAPLSYGSTWLADYWGQGTQVTVSSGGGGSGGGGSQVQLQESGGGLVQAGGSLRLSCAASGRTFSNYNMGWFRQAPGKEREFVAAIDWSGGSPYYAASVRGRFTISRDNAENTVYLQMNSLKPEDTAVYYCAAPLSYGSTWLADYWGQGTQVTVSSEPKSCDKTHTCPPCPAPPVAGPSVFLFPPKPKDTLMISRTPEVTCVVVDVSHEDPEVKFNWYVDGVEVHNAKTKPREEQYNSTYRVVSVLTVLHQDWLNGKEYKCKVSNKGLPSSIEKTISKAKGQPREPQVYTLPPSRDELTKNQVSLSCAVKGFYPSDIAVEWESNGQPENNYKTTPPVLDSDGSFFLVSKLTVDKSRWQQGNVFSCSVMHEALHNHYTQKSLSLSPGK

SEQ ID NO: 158 - protein, 503 aa, synthetic construct
  source 1..503: note = targeting module chain
MGWSCIILFLVATATGVHSGQVQLQESGGGLVQAGGSLRLSCAASGRTFSNYNMGWFRQAPGKEREFVAAIDWSGGSPYYAASVRGRFTISRDNAENTVYLQMNSLKPEDTAVYYCAAPLSYGSTWLADYWGQGTQVTVSSGGGGSGGGGSQVQLQESGGGLVQAGGSLRLSCAASGRTFSNYNMGWFRQAPGKEREFVAAIDWSGGSPYYAASVRGRFTISRDNAENTVYLQMNSLKPEDTAVYYCAAPLSYGSTWLADYWGQGTQVTVSSEPKSCDKTHTCPPCPAPPVAGPSVFLFPPKPKDTLMISRTPEVTCVVVDVSHEDPEVKFNWYVDGVEVHNAKTKPREEQYNSTYRVVSVLTVLHQDWLNGKEYKCKVSNKGLPSSIEKTISKAKGQPREPQVYTLPPSRDELTKNQVSLSCAVKGFYPSDIAVEWESNGQPENNYKTTPPVLDSDGSFFLVSKLTVDKSRWQQGNVFSCSVMHEALHNHYTQKSLSLSPGK

SEQ ID NO: 159 - protein, 484 aa, synthetic construct
  source 1..484: note = targeting module chain
GQVQLVESGGGLVQPGGSLRLSCAASGRTFSNYNMGWFRQAPGQGLEFVAAIDWSGGSPYYADSVKGRFTISRDNSKNTLYLQMNSLRAEDTAVYYCAAPLSYGSTWLADYWGQGTLVTVSSGGGGSGGGGSQVQLVESGGGLVQPGGSLRLSCAASGRTFSNYNMGWFRQAPGQGLEFVAAIDWSGGSPYYADSVKGRFTISRDNSKNTLYLQMNSLRAEDTAVYYCAAPLSYGSTWLADYWGQGTLVTVSSEPKSCDKTHTCPPCPAPPVAGPSVFLFPPKPKDTLMISRTPEVTCVVVDVSHEDPEVKFNWYVDGVEVHNAKTKPREEQYNSTYRVVSVLTVLHQDWLNGKEYKCKVSNKGLPSSIEKTISKAKGQPREPQVYTLPPSRDELTKNQVSLSCAVKGFYPSDIAVEWESNGQPENNYKTTPPVLDSDGSFFLVSKLTVDKSRWQQGNVFSCSVMHEALHNHYTQKSLSLSPGK

SEQ ID NO: 160 - protein, 503 aa, synthetic construct
  source 1..503: note = targeting module chain
MGWSCIILFLVATATGVHSGQVQLVESGGGLVQPGGSLRLSCAASGRTFSNYNMGWFRQAPGQGLEFVAAIDWSGGSPYYADSVKGRFTISRDNSKNTLYLQMNSLRAEDTAVYYCAAPLSYGSTWLADYWGQGTLVTVSSGGGGSGGGGSQVQLVESGGGLVQPGGSLRLSCAASGRTFSNYNMGWFRQAPGQGLEFVAAIDWSGGSPYYADSVKGRFTISRDNSKNTLYLQMNSLRAEDTAVYYCAAPLSYGSTWLADYWGQGTLVTVSSEPKSCDKTHTCPPCPAPPVAGPSVFLFPPKPKDTLMISRTPEVTCVVVDVSHEDPEVKFNWYVDGVEVHNAKTKPREEQYNSTYRVVSVLTVLHQDWLNGKEYKCKVSNKGLPSSIEKTISKAKGQPREPQVYTLPPSRDELTKNQVSLSCAVKGFYPSDIAVEWESNGQPENNYKTTPPVLDSDGSFFLVSKLTVDKSRWQQGNVFSCSVMHEALHNHYTQKSLSLSPGK

SEQ ID NO: 161 - protein, 484 aa, synthetic construct
  source 1..484: note = targeting module chain
GQVQLVESGGGLVQPGGSLRLSCAASGRTFSNYNMGWFRQAPGQGLEFVAAIDWSGGSPYYAASVRGRFTISRDNSKNTLYLQMNSLRAEDTAVYYCAAPLSYGSTWLADYWGQGTLVTVSSGGGGSGGGGSQVQLVESGGGLVQPGGSLRLSCAASGRTFSNYNMGWFRQAPGQGLEFVAAIDWSGGSPYYAASVRGRFTISRDNSKNTLYLQMNSLRAEDTAVYYCAAPLSYGSTWLADYWGQGTLVTVSSEPKSCDKTHTCPPCPAPPVAGPSVFLFPPKPKDTLMISRTPEVTCVVVDVSHEDPEVKFNWYVDGVEVHNAKTKPREEQYNSTYRVVSVLTVLHQDWLNGKEYKCKVSNKGLPSSIEKTISKAKGQPREPQVYTLPPSRDELTKNQVSLSCAVKGFYPSDIAVEWESNGQPENNYKTTPPVLDSDGSFFLVSKLTVDKSRWQQGNVFSCSVMHEALHNHYTQKSLSLSPGK

SEQ ID NO: 162 - protein, 503 aa, synthetic construct
  source 1..503: note = targeting module chain
MGWSCIILFLVATATGVHSGQVQLVESGGGLVQPGGSLRLSCAASGRTFSNYNMGWFRQAPGQGLEFVAAIDWSGGSPYYAASVRGRFTISRDNSKNTLYLQMNSLRAEDTAVYYCAAPLSYGSTWLADYWGQGTLVTVSSGGGGSGGGGSQVQLVESGGGLVQPGGSLRLSCAASGRTFSNYNMGWFRQAPGQGLEFVAAIDWSGGSPYYAASVRGRFTISRDNSKNTLYLQMNSLRAEDTAVYYCAAPLSYGSTWLADYWGQGTLVTVSSEPKSCDKTHTCPPCPAPPVAGPSVFLFPPKPKDTLMISRTPEVTCVVVDVSHEDPEVKFNWYVDGVEVHNAKTKPREEQYNSTYRVVSVLTVLHQDWLNGKEYKCKVSNKGLPSSIEKTISKAKGQPREPQVYTLPPSRDELTKNQVSLSCAVKGFYPSDIAVEWESNGQPENNYKTTPPVLDSDGSFFLVSKLTVDKSRWQQGNVFSCSVMHEALHNHYTQKSLSLSPGK

SEQ ID NO: 163 - protein, 484 aa, synthetic construct
  source 1..484: note = targeting module chain
GQVQLQESGGGLVQAGGSLRLSCAASGRTFSNYNMGWFRQAPGKEREFVAAIDWSGGSPYYAASVRGRFTISRDNAENTVYLQMNSLKPEDTAVYYCAAPLSYGSTWLADYWGQGTQVTVSSGGGGSGGGGSGGGGSEVQLVESGGGLVQPGGSLRLSCAASGFSFSDFWMSWVRQAPGKGLEWVATISQAGSEKDYVDSVKGRFTISRDNAKKSLYLQMNSLRAEDTAVYYCASGVYSFDYRGQGTLVTVSSEPKSCDKTHTCPPCPAPPVAGPSVFLFPPKPKDTLMISRTPEVTCVVVDVSHEDPEVKFNWYVDGVEVHNAKTKPREEQYNSTYRVVSVLTVLHQDWLNGKEYKCKVSNKGLPSSIEKTISKAKGQPREPQVYTLPPSRDELTKNQVSLSCAVKGFYPSDIAVEWESNGQPENNYKTTPPVLDSDGSFFLVSKLTVDKSRWQQGNVFSCSVMHEALHNHYTQKSLSLSPGK

SEQ ID NO: 164 - protein, 503 aa, synthetic construct
  source 1..503: note = targeting module chain
MGWSCIILFLVATATGVHSGQVQLQESGGGLVQAGGSLRLSCAASGRTFSNYNMGWFRQAPGKEREFVAAIDWSGGSPYYAASVRGRFTISRDNAENTVYLQMNSLKPEDTAVYYCAAPLSYGSTWLADYWGQGTQVTVSSGGGGSGGGGSGGGGSEVQLVESGGGLVQPGGSLRLSCAASGFSFSDFWMSWVRQAPGKGLEWVATISQAGSEKDYVDSVKGRFTISRDNAKKSLYLQMNSLRAEDTAVYYCASGVYSFDYRGQGTLVTVSSEPKSCDKTHTCPPCPAPPVAGPSVFLFPPKPKDTLMISRTPEVTCVVVDVSHEDPEVKFNWYVDGVEVHNAKTKPREEQYNSTYRVVSVLTVLHQDWLNGKEYKCKVSNKGLPSSIEKTISKAKGQPREPQVYTLPPSRDELTKNQVSLSCAVKGFYPSDIAVEWESNGQPENNYKTTPPVLDSDGSFFLVSKLTVDKSRWQQGNVFSCSVMHEALHNHYTQKSLSLSPGK

SEQ ID NO: 165 - protein, 484 aa, synthetic construct
  source 1..484: note = targeting module chain
GQVQLVESGGGLVQPGGSLRLSCAASGRTFSNYNMGWFRQAPGQGLEFVAAIDWSGGSPYYADSVKGRFTISRDNSKNTLYLQMNSLRAEDTAVYYCAAPLSYGSTWLADYWGQGTLVTVSSGGGGSGGGGSGGGGSEVQLVESGGGLVQPGGSLRLSCAASGFSFSDFWMSWVRQAPGKGLEWVATISQAGSEKDYVDSVKGRFTISRDNAKKSLYLQMNSLRAEDTAVYYCASGVYSFDYRGQGTLVTVSSEPKSCDKTHTCPPCPAPPVAGPSVFLFPPKPKDTLMISRTPEVTCVVVDVSHEDPEVKFNWYVDGVEVHNAKTKPREEQYNSTYRVVSVLTVLHQDWLNGKEYKCKVSNKGLPSSIEKTISKAKGQPREPQVYTLPPSRDELTKNQVSLSCAVKGFYPSDIAVEWESNGQPENNYKTTPPVLDSDGSFFLVSKLTVDKSRWQQGNVFSCSVMHEALHNHYTQKSLSLSPGK

SEQ ID NO: 166 - protein, 503 aa, synthetic construct
  source 1..503: note = targeting module chain
MGWSCIILFLVATATGVHSGQVQLVESGGGLVQPGGSLRLSCAASGRTFSNYNMGWFRQAPGQGLEFVAAIDWSGGSPYYADSVKGRFTISRDNSKNTLYLQMNSLRAEDTAVYYCAAPLSYGSTWLADYWGQGTLVTVSSGGGGSGGGGSGGGGSEVQLVESGGGLVQPGGSLRLSCAASGFSFSDFWMSWVRQAPGKGLEWVATISQAGSEKDYVDSVKGRFTISRDNAKKSLYLQMNSLRAEDTAVYYCASGVYSFDYRGQGTLVTVSSEPKSCDKTHTCPPCPAPPVAGPSVFLFPPKPKDTLMISRTPEVTCVVVDVSHEDPEVKFNWYVDGVEVHNAKTKPREEQYNSTYRVVSVLTVLHQDWLNGKEYKCKVSNKGLPSSIEKTISKAKGQPREPQVYTLPPSRDELTKNQVSLSCAVKGFYPSDIAVEWESNGQPENNYKTTPPVLDSDGSFFLVSKLTVDKSRWQQGNVFSCSVMHEALHNHYTQKSLSLSPGK

SEQ ID NO: 167 - protein, 484 aa, synthetic construct
  source 1..484: note = targeting module chain
GQVQLVESGGGLVQPGGSLRLSCAASGRTFSNYNMGWFRQAPGQGLEFVAAIDWSGGSPYYAASVRGRFTISRDNSKNTLYLQMNSLRAEDTAVYYCAAPLSYGSTWLADYWGQGTLVTVSSGGGGSGGGGSGGGGSEVQLVESGGGLVQPGGSLRLSCAASGFSFSDFWMSWVRQAPGKGLEWVATISQAGSEKDYVDSVKGRFTISRDNAKKSLYLQMNSLRAEDTAVYYCASGVYSFDYRGQGTLVTVSSEPKSCDKTHTCPPCPAPPVAGPSVFLFPPKPKDTLMISRTPEVTCVVVDVSHEDPEVKFNWYVDGVEVHNAKTKPREEQYNSTYRVVSVLTVLHQDWLNGKEYKCKVSNKGLPSSIEKTISKAKGQPREPQVYTLPPSRDELTKNQVSLSCAVKGFYPSDIAVEWESNGQPENNYKTTPPVLDSDGSFFLVSKLTVDKSRWQQGNVFSCSVMHEALHNHYTQKSLSLSPGK

SEQ ID NO: 168 - protein, 503 aa, synthetic construct
  source 1..503: note = targeting module chain
MGWSCIILFLVATATGVHSGQVQLVESGGGLVQPGGSLRLSCAASGRTFSNYNMGWFRQAPGQGLEFVAAIDWSGGSPYYAASVRGRFTISRDNSKNTLYLQMNSLRAEDTAVYYCAAPLSYGSTWLADYWGQGTLVTVSSGGGGSGGGGSGGGGSEVQLVESGGGLVQPGGSLRLSCAASGFSFSDFWMSWVRQAPGKGLEWVATISQAGSEKDYVDSVKGRFTISRDNAKKSLYLQMNSLRAEDTAVYYCASGVYSFDYRGQGTLVTVSSEPKSCDKTHTCPPCPAPPVAGPSVFLFPPKPKDTLMISRTPEVTCVVVDVSHEDPEVKFNWYVDGVEVHNAKTKPREEQYNSTYRVVSVLTVLHQDWLNGKEYKCKVSNKGLPSSIEKTISKAKGQPREPQVYTLPPSRDELTKNQVSLSCAVKGFYPSDIAVEWESNGQPENNYKTTPPVLDSDGSFFLVSKLTVDKSRWQQGNVFSCSVMHEALHNHYTQKSLSLSPGK

SEQ ID NO: 169 - protein, 483 aa, synthetic construct
  source 1..483: note = targeting module chain
EVQLVESGGGLVQPGGSLRLSCAASGFSFSDFWMSWVRQAPGKGLEWVATISQAGSEKDYVDSVKGRFTISRDNAKKSLYLQMNSLRAEDTAVYYCASGVYSFDYRGQGTLVTVSSEPKSCDKTHTCPPCPAPPVAGPSVFLFPPKPKDTLMISRTPEVTCVVVDVSHEDPEVKFNWYVDGVEVHNAKTKPREEQYNSTYRVVSVLTVLHQDWLNGKEYKCKVSNKGLPSSIEKTISKAKGQPREPQVYTLPPSRDELTKNQVSLSCAVKGFYPSDIAVEWESNGQPENNYKTTPPVLDSDGSFFLVSKLTVDKSRWQQGNVFSCSVMHEALHNHYTQKSLSLSPGKGGGGSGGGGSGGGGSQVQLQESGGGLVQAGGSLRLSCAASGRTFSNYNMGWFRQAPGKEREFVAAIDWSGGSPYYAASVRGRFTISRDNAENTVYLQMNSLKPEDTAVYYCAAPLSYGSTWLADYWGQGTQVTVSS

SEQ ID NO: 170 - protein, 502 aa, synthetic construct
  source 1..502: note = targeting module chain
MGWSCIILFLVATATGVHSEVQLVESGGGLVQPGGSLRLSCAASGFSFSDFWMSWVRQAPGKGLEWVATISQAGSEKDYVDSVKGRFTISRDNAKKSLYLQMNSLRAEDTAVYYCASGVYSFDYRGQGTLVTVSSEPKSCDKTHTCPPCPAPPVAGPSVFLFPPKPKDTLMISRTPEVTCVVVDVSHEDPEVKFNWYVDGVEVHNAKTKPREEQYNSTYRVVSVLTVLHQDWLNGKEYKCKVSNKGLPSSIEKTISKAKGQPREPQVYTLPPSRDELTKNQVSLSCAVKGFYPSDIAVEWESNGQPENNYKTTPPVLDSDGSFFLVSKLTVDKSRWQQGNVFSCSVMHEALHNHYTQKSLSLSPGKGGGGSGGGGSGGGGSQVQLQESGGGLVQAGGSLRLSCAASGRTFSNYNMGWFRQAPGKEREFVAAIDWSGGSPYYAASVRGRFTISRDNAENTVYLQMNSLKPEDTAVYYCAAPLSYGSTWLADYWGQGTQVTVSS

SEQ ID NO: 171 - protein, 483 aa, synthetic construct
  source 1..483: note = targeting module chain
EVQLVESGGGLVQPGGSLRLSCAASGFSFSDFWMSWVRQAPGKGLEWVATISQAGSEKDYVDSVKGRFTISRDNAKKSLYLQMNSLRAEDTAVYYCASGVYSFDYRGQGTLVTVSSEPKSCDKTHTCPPCPAPPVAGPSVFLFPPKPKDTLMISRTPEVTCVVVDVSHEDPEVKFNWYVDGVEVHNAKTKPREEQYNSTYRVVSVLTVLHQDWLNGKEYKCKVSNKGLPSSIEKTISKAKGQPREPQVYTLPPSRDELTKNQVSLSCAVKGFYPSDIAVEWESNGQPENNYKTTPPVLDSDGSFFLVSKLTVDKSRWQQGNVFSCSVMHEALHNHYTQKSLSLSPGKGGGGSGGGGSGGGGSQVQLVESGGGLVQPGGSLRLSCAASGRTFSNYNMGWFRQAPGQGLEFVAAIDWSGGSPYYADSVKGRFTISRDNSKNTLYLQMNSLRAEDTAVYYCAAPLSYGSTWLADYWGQGTLVTVSS

SEQ ID NO: 172 - protein, 502 aa, synthetic construct
  source 1..502: note = targeting module chain
MGWSCIILFLVATATGVHSEVQLVESGGGLVQPGGSLRLSCAASGFSFSDFWMSWVRQAPGKGLEWVATISQAGSEKDYVDSVKGRFTISRDNAKKSLYLQMNSLRAEDTAVYYCASGVYSFDYRGQGTLVTVSSEPKSCDKTHTCPPCPAPPVAGPSVFLFPPKPKDTLMISRTPEVTCVVVDVSHEDPEVKFNWYVDGVEVHNAKTKPREEQYNSTYRVVSVLTVLHQDWLNGKEYKCKVSNKGLPSSIEKTISKAKGQPREPQVYTLPPSRDELTKNQVSLSCAVKGFYPSDIAVEWESNGQPENNYKTTPPVLDSDGSFFLVSKLTVDKSRWQQGNVFSCSVMHEALHNHYTQKSLSLSPGKGGGGSGGGGSGGGGSQVQLVESGGGLVQPGGSLRLSCAASGRTFSNYNMGWFRQAPGQGLEFVAAIDWSGGSPYYADSVKGRFTISRDNSKNTLYLQMNSLRAEDTAVYYCAAPLSYGSTWLADYWGQGTLVTVSS

SEQ ID NO: 173 - protein, 483 aa, synthetic construct
  source 1..483: note = targeting module chain
EVQLVESGGGLVQPGGSLRLSCAASGFSFSDFWMSWVRQAPGKGLEWVATISQAGSEKDYVDSVKGRFTISRDNAKKSLYLQMNSLRAEDTAVYYCASGVYSFDYRGQGTLVTVSSEPKSCDKTHTCPPCPAPPVAGPSVFLFPPKPKDTLMISRTPEVTCVVVDVSHEDPEVKFNWYVDGVEVHNAKTKPREEQYNSTYRVVSVLTVLHQDWLNGKEYKCKVSNKGLPSSIEKTISKAKGQPREPQVYTLPPSRDELTKNQVSLSCAVKGFYPSDIAVEWESNGQPENNYKTTPPVLDSDGSFFLVSKLTVDKSRWQQGNVFSCSVMHEALHNHYTQKSLSLSPGKGGGGSGGGGSGGGGSQVQLVESGGGLVQPGGSLRLSCAASGRTFSNYNMGWFRQAPGQGLEFVAAIDWSGGSPYYAASVRGRFTISRDNSKNTLYLQMNSLRAEDTAVYYCAAPLSYGSTWLADYWGQGTLVTVSS

SEQ ID NO: 174 - protein, 502 aa, synthetic construct
  source 1..502: note = targeting module chain
MGWSCIILFLVATATGVHSEVQLVESGGGLVQPGGSLRLSCAASGFSFSDFWMSWVRQAPGKGLEWVATISQAGSEKDYVDSVKGRFTISRDNAKKSLYLQMNSLRAEDTAVYYCASGVYSFDYRGQGTLVTVSSEPKSCDKTHTCPPCPAPPVAGPSVFLFPPKPKDTLMISRTPEVTCVVVDVSHEDPEVKFNWYVDGVEVHNAKTKPREEQYNSTYRVVSVLTVLHQDWLNGKEYKCKVSNKGLPSSIEKTISKAKGQPREPQVYTLPPSRDELTKNQVSLSCAVKGFYPSDIAVEWESNGQPENNYKTTPPVLDSDGSFFLVSKLTVDKSRWQQGNVFSCSVMHEALHNHYTQKSLSLSPGKGGGGSGGGGSGGGGSQVQLVESGGGLVQPGGSLRLSCAASGRTFSNYNMGWFRQAPGQGLEFVAAIDWSGGSPYYAASVRGRFTISRDNSKNTLYLQMNSLRAEDTAVYYCAAPLSYGSTWLADYWGQGTLVTVSS

SEQ ID NO: 175 - protein, 484 aa, synthetic construct
  source 1..484: note = targeting module chain
DIQLTQSPASLAVSLGQRATISCKASQSVDYDGDSYLNWYQQIPGQPPKLLIYDASNLVSGIPPRFSGSGSGTDFTLNIHPVEKVDAATYHCQQSTEDPWTFGGGTKLEIKGGGGSGGGGSGGGGSGGGGSGGGGSQVQLQQSGAELVRPGSSVKISCKASGYAFSSYWMNWVKQRPGQGLEWIGQIWPGDGDTNYNGKFKGKATLTADESSSTAYMQLSSLASEDSAVYFCARRETTTVGRYYYAMDYWGQGTTVTVSSGGGGSDIVMTQSPDSLAVSLGERATINCKSSQSLLNSRTPKNYLAWYQQKPGQPPKLLIYWASTRKSGVPDRFSGSGSGTDFTLTISSLQAEDVAVYYCKQSYNLLTFGGGTKVEIKRTVAAPSVFIFPPSDEQLKSGTASVVCLLNNFYPREAKVQWKVDNALQSGNSQESVTEQDSKDSTYSLSSTLTLSKADYEKHKVYACEVTHQGLSSPVTKSFNRGEC

SEQ ID NO: 176 - protein, 506 aa, synthetic construct
  source 1..506: note = targeting module chain
MDMRAPAQVFGFLLLWFPGARCDIQLTQSPASLAVSLGQRATISCKASQSVDYDGDSYLNWYQQIPGQPPKLLIYDASNLVSGIPPRFSGSGSGTDFTLNIHPVEKVDAATYHCQQSTEDPWTFGGGTKLEIKGGGGSGGGGSGGGGSGGGGSGGGGSQVQLQQSGAELVRPGSSVKISCKASGYAFSSYWMNWVKQRPGQGLEWIGQIWPGDGDTNYNGKFKGKATLTADESSSTAYMQLSSLASEDSAVYFCARRETTTVGRYYYAMDYWGQGTTVTVSSGGGGSDIVMTQSPDSLAVSLGERATINCKSSQSLLNSRTPKNYLAWYQQKPGQPPKLLIYWASTRKSGVPDRFSGSGSGTDFTLTISSLQAEDVAVYYCKQSYNLLTFGGGTKVEIKRTVAAPSVFIFPPSDEQLKSGTASVVCLLNNFYPREAKVQWKVDNALQSGNSQESVTEQDSKDSTYSLSSTLTLSKADYEKHKVYACEVTHQGLSSPVTKSFNRGEC

SEQ ID NO: 177 - protein, 485 aa, synthetic construct
  source 1..485: note = targeting module chain
GQVQLQQSGAELVRPGSSVKISCKASGYAFSSYWMNWVKQRPGQGLEWIGQIWPGDGDTNYNGKFKGKATLTADESSSTAYMQLSSLASEDSAVYFCARRETTTVGRYYYAMDYWGQGTTVTVSSGGGGSGGGGSGGGGSGGGGSGGGGSDIQLTQSPASLAVSLGQRATISCKASQSVDYDGDSYLNWYQQIPGQPPKLLIYDASNLVSGIPPRFSGSGSGTDFTLNIHPVEKVDAATYHCQQSTEDPWTFGGGTKLEIKGGGGSDIVMTQSPDSLAVSLGERATINCKSSQSLLNSRTPKNYLAWYQQKPGQPPKLLIYWASTRKSGVPDRFSGSGSGTDFTLTISSLQAEDVAVYYCKQSYNLLTFGGGTKVEIKRTVAAPSVFIFPPSDEQLKSGTASVVCLLNNFYPREAKVQWKVDNALQSGNSQESVTEQDSKDSTYSLSSTLTLSKADYEKHKVYACEVTHQGLSSPVTKSFNRGEC

SEQ ID NO: 178 - protein, 504 aa, synthetic construct
  source 1..504: note = targeting module chain
MGWSCIILFLVATATGVHSGQVQLQQSGAELVRPGSSVKISCKASGYAFSSYWMNWVKQRPGQGLEWIGQIWPGDGDTNYNGKFKGKATLTADESSSTAYMQLSSLASEDSAVYFCARRETTTVGRYYYAMDYWGQGTTVTVSSGGGGSGGGGSGGGGSGGGGSGGGGSDIQLTQSPASLAVSLGQRATISCKASQSVDYDGDSYLNWYQQIPGQPPKLLIYDASNLVSGIPPRFSGSGSGTDFTLNIHPVEKVDAATYHCQQSTEDPWTFGGGTKLEIKGGGGSDIVMTQSPDSLAVSLGERATINCKSSQSLLNSRTPKNYLAWYQQKPGQPPKLLIYWASTRKSGVPDRFSGSGSGTDFTLTISSLQAEDVAVYYCKQSYNLLTFGGGTKVEIKRTVAAPSVFIFPPSDEQLKSGTASVVCLLNNFYPREAKVQWKVDNALQSGNSQESVTEQDSKDSTYSLSSTLTLSKADYEKHKVYACEVTHQGLSSPVTKSFNRGEC

SEQ ID NO: 179 - protein, 241 aa, synthetic construct
  source 1..241: note = targeting module chain
MDMRAPAQVFGFLLLWFPGARCDIVMTQSPDSLAVSLGERATINCKSSQSLLNSRTPKNYLAWYQQKPGQPPKLLIYWASTRKSGVPDRFSGSGSGTDFTLTISSLQAEDVAVYYCKQSYNLLTFGGGTKVEIKRTVAAPSVFIFPPSDEQLKSGTASVVCLLNNFYPREAKVQWKVDNALQSGNSQESVTEQDSKDSTYSLSSTLTLSKADYEKHKVYACEVTHQGLSSPVTKSFNRGEC

SEQ ID NO: 180 - protein, 260 aa, synthetic construct
  source 1..260: note = CD19-binding scFv
DIQLTQSPASLAVSLGQRATISCKASQSVDYDGDSYLNWYQQIPGQPPKLLIYDASNLVSGIPPRFSGSGSGTDFTLNIHPVEKVDAATYHCQQSTEDPWTFGGGTKLEIKGGGGSGGGGSGGGGSGGGGSGGGGSQVQLQQSGAELVRPGSSVKISCKASGYAFSSYWMNWVKQRPGQGLEWIGQIWPGDGDTNYNGKFKGKATLTADESSSTAYMQLSSLASEDSAVYFCARRETTTVGRYYYAMDYWGQGTTVTVSS

SEQ ID NO: 181 - protein, 260 aa, synthetic construct
  source 1..260: note = CD19-binding scFv
QVQLQQSGAELVRPGSSVKISCKASGYAFSSYWMNWVKQRPGQGLEWIGQIWPGDGDTNYNGKFKGKATLTADESSSTAYMQLSSLASEDSAVYFCARRETTTVGRYYYAMDYWGQGTTVTVSSGGGGSGGGGSGGGGSGGGGSGGGGSDIQLTQSPASLAVSLGQRATISCKASQSVDYDGDSYLNWYQQIPGQPPKLLIYDASNLVSGIPPRFSGSGSGTDFTLNIHPVEKVDAATYHCQQSTEDPWTFGGGTKLEIK

SEQ ID NO: 182 - protein, 116 aa, synthetic construct
  source 1..116: note = CD19-binding VHH
EVQLVESGGGLVQPGGSLRLSCAASGFSFSDFWMSWVRQAPGKGLEWVATISQAGSEKDYVDSVKGRFTISRDNAKKSLYLQMNSLRAEDTAVYYCASGVYSFDYRGQGTLVTVSS

SEQ ID NO: 183 - protein, 121 aa, Lama glama
  VARIANT 5: note = Xaa can be any naturally occurring amino acid
  VARIANT 14: note = Xaa can be any naturally occurring amino acid
  VARIANT 43: note = Xaa can be any naturally occurring amino acid
  VARIANT 44: note = Xaa can be any naturally occurring amino acid
  VARIANT 45: note = Xaa can be any naturally occurring amino acid
  VARIANT 62: note = Xaa can be any naturally occurring amino acid
  VARIANT 65: note = Xaa can be any naturally occurring amino acid
  VARIANT 75: note = Xaa can be any naturally occurring amino acid
  VARIANT 76: note = Xaa can be any naturally occurring amino acid
  VARIANT 79: note = Xaa can be any naturally occurring amino acid
  VARIANT 87: note = Xaa can be any naturally occurring amino acid
  VARIANT 88: note = Xaa can be any naturally occurring amino acid
  VARIANT 116: note = Xaa can be any naturally occurring amino acid
QVQLXESGGGLVQXGGSLRLSCAASGRTFSNYNMGWFRQAPGXXXEFVAAIDWSGGSPYYAXSVXGRFTISRDNXXNTXYLQMNSLXXEDTAVYYCAAPLSYGSTWLADYWGQGTXVTVSS

SEQ ID NO: 184 - protein, 121 aa, Lama glama
QVQLQESGGGLVQAGGSLRLSCAASGRTFSNYNMGWFRQAPGKEREFVAAIDWSGGSPYYAASVRGRFTISRDNAENTVYLQMNSLKPEDTAVYYCAAPLSYGSTWLADYWGQGTQVTVSS

SEQ ID NO: 185 - protein, 121 aa, synthetic construct
  source 1..121: note = CD20-binding VHH
QVQLVESGGGLVQPGGSLRLSCAASGRTFSNYNMGWFRQAPGQGLEFVAAIDWSGGSPYYADSVKGRFTISRDNSKNTLYLQMNSLRAEDTAVYYCAAPLSYGSTWLADYWGQGTLVTVSS

SEQ ID NO: 186 - protein, 121 aa, synthetic construct
  source 1..121: note = CD20-binding VHH
QVQLVESGGGLVQPGGSLRLSCAASGRTFSNYNMGWFRQAPGQGLEFVAAIDWSGGSPYYAASVRGRFTISRDNSKNTLYLQMNSLRAEDTAVYYCAAPLSYGSTWLADYWGQGTLVTVSS

SEQ ID NO: 187 - protein, 119 aa, Mus musculus
EVQLQQSGPELVKPGASVKMSCKASGYTFTDYYMKWVKQSHGKSLEWIGDIIPSNGATFYNQKFKGKATLTVDRSSSTAYMHLNSLTSEDSAVYYCTRSHLLRASWFAYWGQGTLVTVS

SEQ ID NO: 188 - protein, 113 aa, Mus musculus
DFVMTQSPSSLTVTAGEKVTMSCKSSQSLLNSGNQKNYLTWYLQKPGQPPKLLIYWASTRESGVPDRFTGSGSGTDFTLTISSVQAEDLAVYYCQNDYSYPYTFGGGTKLEIK

SEQ ID NO: 189 - protein, 250 aa, synthetic construct
  source 1..250: note = CD123-binding scFv
EVQLQQSGPELVKPGASVKMSCKASGYTFTDYYMKWVKQSHGKSLEWIGDIIPSNGATFYNQKFKGKATLTVDRSSSTAYMHLNSLTSEDSAVYYCTRSHLLRASWFAYWGQGTLVTVSAASGGGGSGGGGSGGGGSDFVMTQSPSSLTVTAGEKVTMSCKSSQSLLNSGNQKNYLTWYLQKPGQPPKLLIYWASTRESGVPDRFTGSGSGTDFTLTISSVQAEDLAVYYCQNDYSYPYTFGGGTKLEIK

SEQ ID NO: 190 - protein, 526 aa, synthetic construct
  source 1..526: note = targeting module
GQVQLVQSGAEVKKPGSSVKVSCKASGYTFTDYYIHWVRQAPGQGLEWMGDIIPSNGATFYNQRFKGRVTITADESTSTAYMELSSLRSEDTAVYYCTRSHLLRASWFAYWGQGTLVTVSSASGGGGSGGGGSGGGGSDIVMTQTPLSLSVTPGQPASISCRSSQSLLNSGNQKNYLTWYLQKPGQSPQLLIYWASTRFIGVPDRFSGSGSGTDFTLKISRVEAEDVGVYYCQNDYSYPYTFGQGTKLEIKAAARGDIVMTQSPDSLAVSLGERATINCKSSQSLLNSRTPKNYLAWYQQKPGQPPKLLIYWASTRKSGVPDRFSGSGSGTDFTLTISSLQAEDVAVYYCKQSYNLLTFGGGTKVEIKGGGGSGGGGSGASAAGGGGSGGGGSQVQLVQSGAEVKKPGASVKVSCKASGYTFTHYYIYWVRQAPGQGLEWMGGVNPSNGGTHFNEKFKSRVTMTRDTSISTAYMELSRLRSDDTAVYYCARSEYDYGLGFAYWGQGTLVTVSSGGGGSHHHHHHHH

SEQ ID NO: 191 - protein, 526 aa, synthetic construct
  source 1..526: note = targeting module
GQVQLVQSGAEVKKPGASVKMSCKASGYTFTDYYMKWVKQAPGQGLEWIGDIIPSNGATFYNQKFQGRATLTVDTSTSTAYMELSSLRSEDTAVYYCTRSHLLRASWFAYWGQGTLVTVSSASGGGGSGGGGSGGGGSDIVMTQSPDSLAVSLGERATINCKSSQSLLNSGNQKNYLTWYLQKPGQPPKLLIYWASTRESGVPDRFSGSGSGTDFTLTISSVQAEDVAVYYCQNDYSYPYTFGGGTKLEIKAAARGDIVMTQSPDSLAVSLGERVTMNCKSSQSLLNSRTPKNYLAWYQQKPGQSPKLLIYWASTRKSGVPDRFSGSGSGTDFTLTISSVQAEDVAVYYCKQSYNLLTFGGGTKLEIKGGGGSGGGGSGASAAGGGGSGGGGSQVQLVESGAEVVKPGASVKLSCKASGYAFTHYYIYWIKQAPGQGLEWIGGVNPSNGGTHFNEKFKSRATLTVDTSISTAYMELSRLRSDDTAVYYCTRSEYDYGLGFAYWGQGTLVTVSSGGGGSHHHHHHHH

SEQ ID NO: 192 - protein, 525 aa, synthetic construct
  source 1..525: note = targeting module
EVQLQQSGPELVKPGASVKMSCKASGYTFTDYYMKWVKQSHGKSLEWIGDIIPSNGATFYNQKFKGKATLTVDRSSSTAYMHLNSLTSEDSAVYYCTRSHLLRASWFAYWGQGTLVTVSAASGGGGSGGGGSGGGGSDFVMTQSPSSLTVTAGEKVTMSCKSSQSLLNSGNQKNYLTWYLQKPGQPPKLLIYWASTRESGVPDRFTGSGSGTDFTLTISSVQAEDLAVYYCQNDYSYPYTFGGGTKLEIKAAARGDIVMTQSPDSLAVSLGERATINCKSSQSLLNSRTPKNYLAWYQQKPGQPPKLLIYWASTRKSGVPDRFSGSGSGTDFTLTISSLQAEDVAVYYCKQSYNLLTFGGGTKVEIKGGGGSGGGGSGASAAGGGGSGGGGSQVQLVQSGAEVKKPGASVKVSCKASGYTFTHYYIYWVRQAPGQGLEWMGGVNPSNGGTHFNEKFKSRVTMTRDTSISTAYMELSRLRSDDTAVYYCARSEYDYGLGFAYWGQGTLVTVSSGGGGSHHHHHHHH

SEQ ID NO: 193 - protein, 525 aa, synthetic construct
  source 1..525: note = targeting module
EVQLQQSGPELVKPGASVKMSCKASGYTFTDYYMKWVKQSHGKSLEWIGDIIPSNGATFYNQKFKGKATLTVDRSSSTAYMHLNSLTSEDSAVYYCTRSHLLRASWFAYWGQGTLVTVSAASGGGGSGGGGSGGGGSDFVMTQSPSSLTVTAGEKVTMSCKSSQSLLNSGNQKNYLTWYLQKPGQPPKLLIYWASTRESGVPDRFTGSGSGTDFTLTISSVQAEDLAVYYCQNDYSYPYTFGGGTKLEIKAAARGDIVMTQSPDSLAVSLGERVTMNCKSSQSLLNSRTPKNYLAWYQQKPGQSPKLLIYWASTRKSGVPDRFSGSGSGTDFTLTISSVQAEDVAVYYCKQSYNLLTFGGGTKLEIKGGGGSGGGGSGASAAGGGGSGGGGSQVQLVESGAEVVKPGASVKLSCKASGYAFTHYYIYWIKQAPGQGLEWIGGVNPSNGGTHFNEKFKSRATLTVDTSISTAYMELSRLRSDDTAVYYCTRSEYDYGLGFAYWGQGTLVTVSSGGGGSHHHHHHHH

SEQ ID NO: 194 - protein, 526 aa, synthetic construct
  source 1..526: note = targeting module
GQVQLVQSGAEVKKPGASVKMSCKASGYTFTDYYMKWVKQAPGQGLEWIGDIIPSNGATFYNQKFQGRATLTVDTSTSTAYMELSSLRSEDTAVYYCTRSHLLRASWFAYWGQGTLVTVSSASGGGGSGGGGSGGGGSDIVMTQSPDSLAVSLGERATINCKSSQSLLNSGNQKNYLTWYLQKPGQPPKLLIYWASTRESGVPDRFSGSGSGTDFTLTISSVQAEDVAVYYCQNDYSYPYTFGGGTKLEIKAAARGDIVMTQSPDSLAVSLGERATINCKSSQSLLNSRTPKNYLAWYQQKPGQPPKLLIYWASTRKSGVPDRFSGSGSGTDFTLTISSLQAEDVAVYYCKQSYNLLTFGGGTKVEIKGGGGSGGGGSGASAAGGGGSGGGGSQVQLVQSGAEVKKPGASVKVSCKASGYTFTHYYIYWVRQAPGQGLEWMGGVNPSNGGTHFNEKFKSRVTMTRDTSISTAYMELSRLRSDDTAVYYCARSEYDYGLGFAYWGQGTLVTVSSGGGGSHHHHHHHH

SEQ ID NO: 195 - protein, 526 aa, synthetic construct
  source 1..526: note = targeting module
GQVQLVQSGAEVKKPGASVKMSCKASGYTFTDYYMKWVKQAPGQGLEWIGDIIPSNGATFYNQKFKGRATLTVDKSTSTAYMELSSLRSEDTAVYYCTRSHLLRASWFAYWGQGTLVTVSSASGGGGSGGGGSGGGGSDFVMTQSPDSLAVSLGERATMNCKSSQSLLNSGNQKNYLTWYLQKPGQPPKLLIYWASTRESGVPDRFSGSGSGTDFTLTISSVQAEDVAVYYCQNDYSYPYTFGGGTKLEIKAAARGDIVMTQSPDSLAVSLGERATINCKSSQSLLNSRTPKNYLAWYQQKPGQPPKLLIYWASTRKSGVPDRFSGSGSGTDFTLTISSLQAEDVAVYYCKQSYNLLTFGGGTKVEIKGGGGSGGGGSGASAAGGGGSGGGGSQVQLVQSGAEVKKPGASVKVSCKASGYTFTHYYIYWVRQAPGQGLEWMGGVNPSNGGTHFNEKFKSRVTMTRDTSISTAYMELSRLRSDDTAVYYCARSEYDYGLGFAYWGQGTLVTVSSGGGGSHHHHHHHH

SEQ ID NO: 196 - protein, 525 aa, synthetic construct
  source 1..525: note = targeting module
EVQLVQSGAEVKKPGASVKMSCKASGYTFTDYYMKWVKQAPGQGLEWIGDIIPSNGATFYNQKFKGRATLTVDRSTSTAYMELSSLRSEDTAVYYCTRSHLLRASWFAYWGQGTLVTVSSASGGGGSGGGGSGGGGSDFVMTQSPDSLAVSLGERATINCESSQSLLNTGNQKNYLTWYLQKPGQPPKLLIYWASTRESGVPDRFSGSGSGTDFTLTISSVQAEDVAVYYCQNDYSYPYTFGGGTKLEIKAAARGDIVMTQSPDSLAVSLGERATINCKSSQSLLNSRTPKNYLAWYQQKPGQPPKLLIYWASTRKSGVPDRFSGSGSGTDFTLTISSLQAEDVAVYYCKQSYNLLTFGGGTKVEIKGGGGSGGGGSGASAAGGGGSGGGGSQVQLVQSGAEVKKPGASVKVSCKASGYTFTHYYIYWVRQAPGQGLEWMGGVNPSNGGTHFNEKFKSRVTMTRDTSISTAYMELSRLRSDDTAVYYCARSEYDYGLGFAYWGQGTLVTVSSGGGGSHHHHHHHH

SEQ ID NO: 197 - protein, 525 aa, synthetic construct
  source 1..525: note = targeting module
EVQLVQSGAEVKKPGASVKMSCKASGYTFTDYYMKWVKQAPGQGLEWIGDIIPSNGATFYNQKFKGRATLTVDRSTSTAYMELSSLRSEDTAVYYCTRSHLLRASWFAYWGQGTLVTVSSASGGGGSGGGGSGGGGSDFVMTQSPDSLAVSLGERATINCESSQSLLNTGNQKNYLTWYLQKPGQPPKLLIYWASTRESGVPDRFSGSGSGTDFTLTISSVQAEDVAVYYCQNDYSYPYTFGGGTKLEIKAAARGDIVMTQSPDSLAVSLGERVTMNCKSSQSLLNSRTPKNYLAWYQQKPGQSPKLLIYWASTRKSGVPDRFSGSGSGTDFTLTISSVQAEDVAVYYCKQSYNLLTFGGGTKLEIKGGGGSGGGGSGASAAGGGGSGGGGSQVQLVESGAEVVKPGASVKLSCKASGYAFTHYYIYWIKQAPGQGLEWIGGVNPSNGGTHFNEKFKSRATLTVDTSISTAYMELSRLRSDDTAVYYCTRSEYDYGLGFAYWGQGTLVTVSSGGGGSHHHHHHHH